European Patent Application EP 4 772 626 A1, published July 8, 2026. Title: ゲノム編集技術. Applicant: 学校法人　関西大学. The sequence listing filed with the application follows.

SEQUENCE LISTING (78 sequences)

SEQ ID NO: 1 - DNA, 1560 bp, synthetic construct
  source 1..1560: mol_type = other DNA
  misc_feature 1..1560: note = PermE-codAsm
attcgatatcatgtcggaccggagttcgaggtacgcggcttgcaggtccaggaaggggacgtccatgcgagtgtccgttcgagtggcggcttgcgcccgatgctagtcgcggttgatcggcgatcgcaggtgcacgcggtcgatcttgacggctggcgagaggtgcggggaggatctgaccgacgcggtccacacgtggcaccgcgatgctgttgtgggcacaatcgtgccggttggtaggatcctcgaggacaggaggctgccatatgccgaacaacgcgcttcagacgatcatcaacgcccgcctgcccggtgaggaaggcctgtggcaaatccacctgcaagacggcaagatctcggccatcgacgcccagtccggagtgatgccgatcacggagaacagcctggacgcggagcagggcctggtgatccccccgttcgtcgagccccacatccacttggacaccacccagacggccggccagcccaactggaaccagtcgggcaccctgttcgagggcatcgagcggtgggccgagcgcaaggcgctgctgacccacgacgacgtgaagcagcgggcgtggcagaccctcaagtggcagatcgccaacggcatccagcacgtacgcacgcacgtggacgtctccgatgcgaccctcacggccctgaaggccatgctcgaagtcaagcaggaggtggccccgtggatcgacctccagatcgtcgccttcccgcaggagggcatcctctcgtaccccaacggcgaagccctcctggaggaggccctgcggctgggagccgacgtcgtcggtgccatcccgcacttcgagttcacccgcgagtacggcgttgagagcctgcacaagaccttcgcgctggcgcagaagtacgaccgcctgatcgacgtccactgcgacgagatcgacgacgagcagtcccggttcgtggagaccgtcgcggcactggcccatcacgagggcatgggtgcccgcgtcacagcgtcccacaccacggccatgcactcctacaacggcgcctacacctcccgcctgttccgcctcctgaagatgtcgggcatcaacttcgtcgccaatcccctcgtgaacatccacctccagggcaggttcgacacgtacccgaaacggcggggcattacccgcgtcaaggagatgctcgaatcggggatcaacgtgtgcttcgggcacgcggacgtcttcgacccgtggtacccgctcggcaccgccaacatgctccaggtcctgcacatgggcctgcacgtctgccagctgatgggctacgggcagatcaacgacgggctgaacctcatcacgcaccacagtgcccgtaccctgaacctccaggactacggcatcgccgctgggaactccgccaacctgatcatcctgccagcggagaacggcttcgacgcgctccgtcggcaggtgccggtgcgctacagcgtccgaggcggcaaggtcatcgcgagcacccagcccgcacagaccaccgtctatctggagcagccggaggcgatcgactacaagcgctgatctagagtcg

SEQ ID NO: 2 - DNA, 37 bp, synthetic construct
  source 1..37: mol_type = other DNA
  misc_feature 1..37: note = codA-hindF
ggcatgcaagcttattcgatatcatgtcggaccggag

SEQ ID NO: 3 - DNA, 34 bp, synthetic construct
  source 1..34: mol_type = other DNA
  misc_feature 1..34: note = codA-nheR
gcgtgaagctagctcagcgcttgtagtcgatcgc

SEQ ID NO: 4 - DNA, 47 bp, synthetic construct
  source 1..47: mol_type = other DNA
  misc_feature 1..47: note = p15A ori-F
atctcatgaccaaaatcccttaattaagtgcgtcgggtgatgctgcc

SEQ ID NO: 5 - DNA, 44 bp, synthetic construct
  source 1..44: mol_type = other DNA
  misc_feature 1..44: note = p15A ori-R
tgagtgagctaactcacattaatttaactgtgataaactaccgc

SEQ ID NO: 6 - DNA, 5379 bp, synthetic construct
  source 1..5379: mol_type = other DNA
  misc_feature 1..5379: note = pPacI-int
atctcatgaccaaaatcccttaattaagtgcgtcgggtgatgctgccaacttactgatttagtgtatgatggtgtttttgaggtgctccagtggcttctgtttctatcagctgtccctcctgttcagctactgacggggtggtgcgtaacggcaaaagcaccgccggacatcagcgctagcggagtgtatactggcttactatgttggcactgatgagggtgtcagtgaagtgcttcatgtggcaggagaaaaaaggctgcaccggtgcgtcagcagaatatgtgatacaggatatattccgcttcctcgctcactgactcgctacgctcggtcgttcgactgcggcgagcggaaatggcttacgaacggggcggagatttcctggaagatgccaggaagatacttaacagggaagtgagagggccgcggcaaagccgtttttccataggctccgcccccctgacaagcatcacgaaatctgacgctcaaatcagtggtggcgaaacccgacaggactataaagataccaggcgtttccccctggcggctccctcgtgcgctctcctgttcctgcctttcggtttaccggtgtcattccgctgttatggccgcgtttgtctcattccacgcctgacactcagttccgggtaggcagttcgctccaagctggactgtatgcacgaaccccccgttcagtccgaccgctgcgccttatccggtaactatcgtcttgagtccaacccggaaagacatgcaaaagcaccactggcagcagccactggtaattgatttagaggagttagtcttgaagtcatgcgccggttaaggctaaactgaaaggacaagttttggtgactgcgctcctccaagccagttacctcggttcaaagagttggtagctcagagaaccttcgaaaaaccgccctgcaaggcggttttttcgttttcagagcaagagattacgcgcagaccaaaacgatctcaagaagatcatcttattaatcagataaaatatttctagatttcagtgcaatttatctcttcaaatgtagcacctgaagtcagccccatacgatataagttgtaattctcatgtttgacagcttatcatcgataagctttaatgcggtagtttatcacagttaaattaatgtgagttagctcactcattaggcaccccaggctttacactttatgcttccggctcgtatgttgtgtggaattgtgagcggataacaatttcacacaggaaacagctatgaccatgattacgaattcgagctcggtacccggggatcctctagagtcgacctgcaggcatgcaagcttattcgatatcatgtcggaccggagttcgaggtacgcggcttgcaggtccaggaaggggacgtccatgcgagtgtccgttcgagtggcggcttgcgcccgatgctagtcgcggttgatcggcgatcgcaggtgcacgcggtcgatcttgacggctggcgagaggtgcggggaggatctgaccgacgcggtccacacgtggcaccgcgatgctgttgtgggcacaatcgtgccggttggtaggatcctcgaggacaggaggctgccatatgccgaacaacgcgcttcagacgatcatcaacgcccgcctgcccggtgaggaaggcctgtggcaaatccacctgcaagacggcaagatctcggccatcgacgcccagtccggagtgatgccgatcacggagaacagcctggacgcggagcagggcctggtgatccccccgttcgtcgagccccacatccacttggacaccacccagacggccggccagcccaactggaaccagtcgggcaccctgttcgagggcatcgagcggtgggccgagcgcaaggcgctgctgacccacgacgacgtgaagcagcgggcgtggcagaccctcaagtggcagatcgccaacggcatccagcacgtacgcacgcacgtggacgtctccgatgcgaccctcacggccctgaaggccatgctcgaagtcaagcaggaggtggccccgtggatcgacctccagatcgtcgccttcccgcaggagggcatcctctcgtaccccaacggcgaagccctcctggaggaggccctgcggctgggagccgacgtcgtcggtgccatcccgcacttcgagttcacccgcgagtacggcgttgagagcctgcacaagaccttcgcgctggcgcagaagtacgaccgcctgatcgacgtccactgcgacgagatcgacgacgagcagtcccggttcgtggagaccgtcgcggcactggcccatcacgagggcatgggtgcccgcgtcacagcgtcccacaccacggccatgcactcctacaacggcgcctacacctcccgcctgttccgcctcctgaagatgtcgggcatcaacttcgtcgccaatcccctcgtgaacatccacctccagggcaggttcgacacgtacccgaaacggcggggcattacccgcgtcaaggagatgctcgaatcggggatcaacgtgtgcttcgggcacgcggacgtcttcgacccgtggtacccgctcggcaccgccaacatgctccaggtcctgcacatgggcctgcacgtctgccagctgatgggctacgggcagatcaacgacgggctgaacctcatcacgcaccacagtgcccgtaccctgaacctccaggactacggcatcgccgctgggaactccgccaacctgatcatcctgccagcggagaacggcttcgacgcgctccgtcggcaggtgccggtgcgctacagcgtccgaggcggcaaggtcatcgcgagcacccagcccgcacagaccaccgtctatctggagcagccggaggcgatcgactacaagcgctgatctagagtcggctagcttcacgctgccgcaagcactcagggcgcaagggctgctaaaggaagcggaacacgtagaaagccagtccgcagaaacggtgctgaccccggatgaatgtcagctactgggctatctggacaagggaaaacgcaagcgcaaagagaaagcaggtagcttgcagtgggcttacatggcgatagctagactgggcggttttatggacagcaagcgaaccggaattgccagctggggcgccctctggtaaggttgggaagccctgcaaagtaaactggatggctttcttgccgccaaggatctgatggcgcaggggatcaagatctgatcaagagacaggatgaggatcgtttcgcatgattgaacaagatggattgcacgcaggttctccggccgcttgggtggagaggctattcggctatgactgggcacaacagacaatcggctgctctgatgccgccgtgttccggctgtcagcgcaggggcgcccggttctttttgtcaagaccgacctgtccggtgccctgaatgaactccaagacgaggcagcgcggctatcgtggctggccacgacgggcgttccttgcgcagctgtgctcgacgttgtcactgaagcgggaagggactggctgctattgggcgaagtgccggggcaggatctcctgtcatctcaccttgctcctgccgagaaagtatccatcatggctgatgcaatgcggcggctgcatacgcttgatccggctacctgcccattcgaccaccaagcgaaacatcgcatcgagcgagcacgtactcggatggaagccggtcttgtcgatcaggatgatctggacgaagagcatcaggggctcgcgccagccgaactgttcgccaggctcaaggcgcggatgcccgacggcgaggatctcgtcgtgacccatggcgatgcctgcttgccgaatatcatggtggaaaatggccgcttttctggattcatcgactgtggccggctgggtgtggcggaccgctatcaggacatagcgttggctacccgtgatattgctgaagagcttggcggcgaatgggctgaccgcttcctcgtgctttacggtatcgccgctcccgattcgcagcgcatcgccttctatcgccttcttgacgagttcttctgagcgggactctggggttcgaaatgaccgaccaagcgacgcccaacctgccatcacgagatttcgattccaccgccgccttctatgaaaggttgggcttcggaatcgttttccgggacgccctcgcggacgtgctcatagtccacgacgcccgtgattttgtagccctggccgacggccagcaggtaggccgacaggctcatgccggccgccgccgccttttcctcaatcgctcttcgttcgtctggaaggcagtacaccttgataggtgggctgcccttcctggttggcttggtttcatcagccatccgcttgccctcatctgttacgccggcggtagccggccagcctcgcagagcaggattcccgttgagcaccgccaggtgcgaataagggacagtgaagaaggaacacccgctcgcgggtgggcctacttcacctatcctgccccgctgacgccgttggatacaccaaggaaagtctacacgaaccctttggcaaaatcctgtatatcgtgcgaaaaaggatggatataccgaaaaaatcgctataatgaccccgaagcagggttatgcagcggaaaagcgctgcttccctgctgttttgtggaatatctaccgactggaaacaggcaaatgcaggaaattactgaactgaggggacaggcgagagacgatgccaaagagctcctgaaaatctcgataactcaaaaaatacgcccggtagtgatcttatttcattatggtgaaagttggaacctcttacgtgccgatcaacgtctcattttcgccaaaagttggcccagggcttcccggtatcaacagggacaccaggatttatttattctgcgaagtgatcttccgtcacaggtatttattcggcgcaaagtgcgtcgggtgatgctgccaacttactgatttagtgtatgatggtgtttttgaggtgctccagtggcttctgtttctatcagctcctgaaaatctcgataactcaaaaaatacgcccggtagtgatcttatttcattatggtgaaagttggaacctcttacgtgccgatcaacgtctcattttcgccaaaagttggcccagggcttcccggtatcaacagggacaccaggatttatttattctgcgaagtgatcttccgtcacaggtatttattcggcgcaaagtgcgtcgggtgatgctgccaacttactgatttagtgtatgatggtgtttttgaggtgctccagtggcttctgtttctatcagggctggatgatcctccagcgcggggatctcatgctggagttcttcgcccaccccaaaaggatctaggtgaagatcctttttgata

SEQ ID NO: 7 - DNA, 176 bp, synthetic construct
  source 1..176: mol_type = other DNA
  misc_feature 1..176: note = PtipA
tatgacatgattacgaattcgatatcagggctacgctggaccggatgggctgagggagccgacggcacgcggcggctcacggcgtggcacgcggaacgtccgggcttgcacctcacgtcacgtgaggaggcagcgtggacggcgtcagagaagggagcggagcatatgagcaaggg

SEQ ID NO: 8 - DNA, 54 bp, synthetic construct
  source 1..54: mol_type = other DNA
  misc_feature 1..54: note = PtipA-EcoRV-1F
tatgacatgattacgaattcgatatcagggctacgctggaccggatgggctgag

SEQ ID NO: 9 - DNA, 64 bp, synthetic construct
  source 1..64: mol_type = other DNA
  misc_feature 1..64: note = PtipA-2R
cgttccgcgtgccacgccgtgagccgccgcgtgccgtcggctccctcagcccatccggtccagc

SEQ ID NO: 10 - DNA, 64 bp, synthetic construct
  source 1..64: mol_type = other DNA
  misc_feature 1..64: note = PtipA-3F
acggcgtggcacgcggaacgtccgggcttgcacctcacgtcacgtgaggaggcagcgtggacgg

SEQ ID NO: 11 - DNA, 55 bp, synthetic construct
  source 1..55: mol_type = other DNA
  misc_feature 1..55: note = PtipA-NdeI-4R
cccttgctcatatgctccgctcccttctctgacgccgtccacgctgcctcctcac

SEQ ID NO: 12 - DNA, 717 bp, synthetic construct
  source 1..717: mol_type = other DNA
  misc_feature 1..717: note = gfpuv (codon optimized)
atgagcaagggcgaggagctgttcaccggcgtggtgccgatcctggtcgaactggacggggacgtcaacggccacaagttctcggtgtccggtgagggcgaaggcgacgccacgtacggcaagctcaccctgaagttcatctgcacgacgggcaagctgcccgtgccctggcccacgctcgtcacgaccttcagctacggcgtccagtgcttctcgcgctacccggaccacatgaagcggcacgacttcttcaagtccgccatgccggagggctacgtccaggaacgcaccatctccttcaaggacgacggcaactacaagacccgcgcggaggtcaagttcgagggcgacaccctggtcaaccgcatcgagctgaagggcatcgacttcaaggaggacggcaacatcctgggccacaagctcgagtacaactacaactcccacaacgtctacatcaccgccgacaagcagaagaacgggatcaaggcgaacttcaagatccggcacaacatcgaggacggctccgtgcagctggccgaccactaccagcagaacaccccgatcggcgacggtccggtcctgctgcccgacaaccactacctctccacccagtcggccctgtcgaaggacccgaacgagaagcgcgaccacatggtcctcctggagttcgtgaccgcggccgggatcacccacgggatggacgagctctacaagtga

SEQ ID NO: 13 - DNA, 29 bp, synthetic construct
  source 1..29: mol_type = other DNA
  misc_feature 1..29: note = gfp-ndeF
gcggagcatatgagcaagggcgaggagct

SEQ ID NO: 14 - DNA, 44 bp, synthetic construct
  source 1..44: mol_type = other DNA
  misc_feature 1..44: note = gfp-kpnR
tggagatctagcggtaccggctcacttgtagagctcgtccatcc

SEQ ID NO: 15 - DNA, 7875 bp, synthetic construct
  source 1..7875: mol_type = other DNA
  misc_feature 1..7875: note = pLAE001
tcgcgcgtttcggtgatgacggtgaaaacctctgacacatgcagctcccggagacggtcacagcttgtctgtaagcggatgccgggagcagacaagcccgtcagggcgcgtcagcgggtgttggcgggtgtcggggctggcttaactatgcggcatcagagcagattgtactgagagtgcaccatatgcggtgtgaaataccgcacagatgcgtaaggagaaaataccgcatcaggcgccattcgccattcaggctgcgcaactgttgggaagggcgatcggtgcgggcctcttcgctattacgccagctggcgaaagggggatgtgctgcaaggcgattaagttgggtaacgccagggttttcccagtcacgacgttgtaaaacgacggccagtgaattcgagctcggtacccgggggcgcgccggatccttaattaagtctagagtcgactgtttaaacctgcaggcatgcaagcttggcgtaatcatggtcatagctgtttcctgtgtgaaattgttatccgctcacaattccacacaacatacgagccggaagcataaagtgtaaagcctggggtgcctaatgagtgagctaactcacattaattgcgttgcgctcactgcccgctttccagtcgggaaacctgtcgtgccagctgcattaatgaatcggccaacgcgcggggagaggcggtttgcgtattgggcgctcttccgcttcctcgctcactgactcgctgcgctcggtcgttcggctgcggcgagcggtatcagctcactcaaaggcggtaatacggttatccacagaatcaggggataacgcaggaaagaacatgtgagcaaaaggccagcaaaaggccaggaaccgtaaaaaggccgcgttgctggcgtttttccataggctccgcccccctgacgagcatcacaaaaatcgacgctcaagtcagaggtggcgaaacccgacaggactataaagataccaggcgtttccccctggaagctccctcgtgcgctctcctgttccgaccctgccgcttaccggatacctgtccgcctttctcccttcgggaagcgtggcgctttctcatagctcacgctgtaggtatctcagttcggtgtaggtcgttcgctccaagctgggctgtgtgcacgaaccccccgttcagcccgaccgctgcgccttatccggtaactatcgtcttgagtccaacccggtaagacacgacttatcgccactggcagcagccactggtaacaggattagcagagcgaggtatgtaggcggtgctacagagttcttgaagtggtggcctaactacggctacactagaagaacagtatttggtatctgcgctctgctgaagccagttaccttcggaaaaagagttggtagctcttgatccggcaaacaaaccaccgctggtagcggtggtttttttgtttgcaagcagcagattacgcgcagaaaaaaaggatctcaagaagatcctttgatcttttctacggggtctgacgctcagtggaacgaaaactcacgttaagggattttggtcatgagattatcaaaaaggatcttcacctagatccttttaaattaaaaatgaagttttaaatcaatctaaagtatatatgagtaaacttggtctgacagttaccaatgcttaatcagtgaggcacctatctcagcgatctgtctatttcgttcatccatagttgcctgactccccgtcgtgtagataactacgatacgggagggcttaccatctggccccagtgctgcaatgataccgcgagacccacgctcaccggctccagatttatcagcaataaaccagccagccggaagggccgagcgcagaagtggtcctgcaactttatccgcctccatccagtctattaattgttgccgggaagctagagtaagtagttcgccagttaatagtttgcgcaacgttgttgccattgctacaggcatcgtggtgtcacgctcgtcgtttggtatggcttcattcagctccggttcccaacgatcaaggcgagttacatgatcccccatgttgtgcaaaaaagcggttagctccttcggtcctccgatcgttgtcagaagtaagttggccgcagtgttatcactcatggttatggcagcactgcataattctcttactgtcatgccatccgtaagatgcttttctgtgactggtgagtactcaaccaagtcattctgagaatagtgtatgcggcgaccgagttgctcttgcccggcgtcaatacgggataataccgcgccacatagcagaactttaaaagtgctcatcattggaaaacgttcttcggggcgaaaactctcaaggatcttaccgctgttgagatccagttcgatgtaacccactcgtgcacccaactgatcttcagcatcttttactttcaccagcgtttctgggtgagcaaaaacaggaaggcaaaatgccgcaaaaaagggaataagggcgacacggaaatgttgaatactcatactcttcctttttcaatattattgaagcatttatcagggttattgtctcatgagcggatacatatttgaatgtatttagaaaaataaacaaataggggttccgcgcacatttccccgaaaagtgccacctgcagatcaaggcgaatacttcatatgcggggatcgaccgcgcgggtcccggacggggaagagcggggagctttgccagagagcgacgacttccccttgcgttggtgattgccggtcagggcagccatccgccatcgtcgcgtagggtgtcacaccccaggaatcgcgtcactgaacacagcagccggtaggacgaccatgactgagttggacaccatcgcaaatccgtccgatcccgcggtgcagcggatcatcgatgtcaccaagccgtcgcgatccaacataaagacaacgttgatcgaggacgtcgagcccctcatgcacagcatcgcggccggggtggagttcatcgaggtctacggcagcgacagcagtccttttccatctgagttgctggatctgtgcgggcggcagaacataccggtccgcctcatcgactcctcgatcgtcaaccagttgttcaagggggagcggaaggccaagacattcggcatcgcccgcgtccctcgcccggccaggttcggcgatatcgcgagccggcgtggggacgtcgtcgttctcgacggggtgaagatcgtcgggaacatcggcgcgatagtacgcacgtcgctcgcgctcggagcgtcggggatcatcctggtcgacagtgacatcaccagcatcgcggaccggcgtctccaaagggccagccgaggttacgtcttctcccttcccgtcgttctctccggtcgcgaggaggccatcgccttcattcgggacagcggtatgcagctgatgacgctcaaggcggatggcgacatttccgtgaaggaactcggggacaatccggatcggctggccttgctgttcggcagcgaaaagggtgggccttccgacctgttcgaggaggcgtcttccgcctcggtttccatccccatgatgagccagaccgagtctctcaacgtttccgtttccctcggaatcgcgctgcacgagaggatcgacaggaatctcgcggccaaccgataagcgcctctgttcctcggacgctcggttcctcgacctcgattcgtcagtgatgatcctgtgctttggtctctgacatgcccttagtctagcagtttctgacttactgtttccagaaagtcagaaactaaaaactggcaactcgctgcgaatctcggggggttcggtttccgggccggccggtcggtcggcccgctcgcggggcgggtgcttcgtcggtccctgcggcccggtggcccgtccggtctcggcggcgggctatgcccagcacgctggccgttcgcgtgtacacacatcacgcggtgcggggcctgcactccgccggcgggtgttcgccgctgcgggtttcggtcggctcctcggactcgcctgctcagtccgtggtgatctgtcgccgtcctgtggtgcctactgtagcgcctcgggtgccctcccgtggcgcggttcaccctttgggtgtgtcggcgcgtcctgcggggcctccacggcctcaggcggcgagcgtgatcgtgccgggctccgccgcggtgggccggtggccggcgagtcgggcggggtcgatgacctcgccgcgctgcgcaagggtggtggcctcggcggcgagttcggcggcgccgatccgggcggcctcgatggcgaacgcgcgggagtggtcggcggctccgggctgtcccagctcggtgggggcctggcgggggtaggcgcgggcgtacgggtccaggccggggagaaccgcttggtcggcgctggcccgggggcctcggcttcggcgctcgtcgcggtcgagctgccaccacgcctcttctcggcaccaccactggtgttggctctgctcgactcgggccaccacggcgagttccacgggacggctggccactcccaccgcggccccggcctcgtacaggctccggtccgtcggcacgagggcgccctcagcggtgatctccgccaagccggcctccaccagcctgccgcagtgccgggcggtcgtacgggccgtgtagccgctgtgctgggtgatctcctccgggctcacgccggccgggtggtccttgatgatctccagcgtgcgggccgcgtggtgcccgaaccggtgccagatacccgcctgctgatgggcaaccaatcctccgagacggccaaggactcccaccccgcccctgggggggcggggtgttccgcttctgtccgacccgtggtgacctgctgttttgctgtctgctggcaggtcgtgaagggcgcacatgtggtgctcgtcggcggtgcactggtgggcgcgggccagccggatgcggcggccactgctggtgcggcgctcggcgtccttcgcggtctcgatccacccgtcgtaggtgacgcgttgcagggacagtgcggccgtggacttggagtagccggcgagtacggcgatccggcggacgctggcggtcacctcgaccagcccgtaggcggccatgaaccatgcgagcgcgcgcaacacggcgcggtcggcggggccgctgggcctggtccagtgggcgtgcccgcacgcctccatgcgggcgatcaggtcggtggcagcggccatgccctcggcggcgccttgctgctcgtcgtcctggtcggtctccgcgcggcggtggggcatccgggcggcgtcctgcaccgcgagccaccacgcgcgggtgagccggtcctcggcctccgcctcggtgagcggggcacgctcgccggtggcggtgctggcggtgcgcaaccactccagcgccggggacaactcggggtcggcggcgaacgcggcggcctcgccgcggtgccacccggcggcggccatggaccgcaaaacggggtgtacggccgcctggtgggcgccgggggtgctgctggggcggtgctcggcgccgcgtcgggcggcgccgctcaggaggcgccagggcacgtccagccggggcacaccgccctcgtcggtcacgaccggccgcaccaccgggccgcgggccgcgatggacggcggaaccgaccggccgccgctcccaccgcggcgtgcccgggactcgccgagtgccgcatccgccacgcgccacaagccggccgccttcgcctgggcctccagatcgcgcagcagcgccacgaacgcgcgggcctgggcaccctgcttgaggaccgcgaccgcttcctcgacactgtgccggacaagttcggcgtacccgccgtggcggtgcggagcgccggggggcctgacggctccgctggcggggttcaacagcggcgtgcggtccaccgtcgggaacagggcctgggccgcatccgcgatccgggccaccaccaccggcggcaagccctgcggacacgccacccacacgtgcatgcccccgctcggaccggagttgaccggcaccgcgccgatgccgtgcgctgccagcaactcgaccagggcggcggcgtgacggcgtaccgcctcccgtccgcccctcgacacgtccagctcgaacacgacgtacacgtaaacgtggtagcggtcgctgcggcgcccacccttgcggttgcggaaaccggtcaaatacatcgcgaccggcgccgacccgtccacctcgtcccggtcgatgacaaccggatacgagttagcccaaacagtggcggaattctcctgtacacgcgaactgtcgtcgccgatgaactgcgctcgccgcaccttccggctcggcgacaactcccggagaaaccgggacaaaacatctcgatgcgatgcggtggcagtgtcgacaaatcgcccctcagacaccccggattgaggcaaagaggtaccgccaccgtggctctgcgctacgatggcgacagctcctcggtgctaagaggacgcacagacgcccccgctcgtcggcctaggaaaccggcacaaacggcggctgatgtgctttttctggggcccggagtctcagcggtggttggggaacctgaaggtgctgggacccggggggacctggggcttacgtacgcgcttcggttaggaagtccgaagcgcccttacgcgcgcccgttccttcaactggcctccttgagctgtgctgcggacggccatcccataggcccacccgtttgggggtctacctccaccacgcctactagggcgttgaggaacccggcgacggacatgttcagcgcggcgcacatgtcgatgagcttcatggcgttgtccggctcaaaacctgttcctgggcggtagggaccaccgctcgccgggtcgtaggacggagcacggtaccgggtaccgcgcggcatcccgcgacgccgcggttgctgatccttttccatggtcaaggatcatgccacaaaagtgcagcaccagggaggagaattgctgcactttccctcggcgtgttgaaagttcccccgccaaaagccccttaagggatattgcactcgttctgacttgacgcgacgcctgtcaccgtgctggcccctgaggctgactagtcgtcttcttcgccgtcagggtcgatgggctcggcgggggtgaagggggatgcgcatgcgtggcagtgcaatccgccgtcttctccgccggccatccatgccttgcggctgatctggatgcggcgggcgggctggagttcgccgtctttgccctcctcggtgcactggcaggtgatgaggaatcgggtgttcccccgcttcttcttcggcctgacggggccctcctgcgggtcctggtcctcgtcctcgtcctcgccgtcctcgcctgccgtggcggtgccggggtcggcgccgccgatcaagagggcaagggggtcgtggaggtaggggagttgggcttggtccagggcctcgatggcggcggcgtacttggccgcggtggcatccgtgatggtgcactcgttccagccgttgactgggacgctcgcggcggggccggcgagtcccagttcctccgcgacggccacgaaacgcctgttgtggtagcggccatcgctgctggtgtcggcgatccgccggacgtgcgcgacggcgtgtgcggcctcgtgcagcagcgtttgcatcgtcctgcgtccgccgagtgccaacagctcgccgccggcgaacagctcgggggccttgcggcggccggcgcccttgagggtccacatgtcggcaccgaagtgaccccacttgatgctccgggcgctgcggccggtgccggtgatctgctaagaaaccattattatcatgacattaacctataaaaataggcgtatcacgaggccctttcgtc

SEQ ID NO: 16 - DNA, 810 bp, synthetic construct
  source 1..810: mol_type = other DNA
  misc_feature 1..810: note = tsr
atgactgagttggacaccatcgcaaatccgtccgatcccgcggtgcagcggatcatcgatgtcaccaagccgtcgcgatccaacataaagacaacgttgatcgaggacgtcgagcccctcatgcacagcatcgcggccggggtggagttcatcgaggtctacggcagcgacagcagtccttttccatctgagttgctggatctgtgcgggcggcagaacataccggtccgcctcatcgactcctcgatcgtcaaccagttgttcaagggggagcggaaggccaagacattcggcatcgcccgcgtccctcgcccggccaggttcggcgatatcgcgagccggcgtggggacgtcgtcgttctcgacggggtgaagatcgtcgggaacatcggcgcgatagtacgcacgtcgctcgcgctcggagcgtcggggatcatcctggtcgacagtgacatcaccagcatcgcggaccggcgtctccaaagggccagccgaggttacgtcttctcccttcccgtcgttctctccggtcgcgaggaggccatcgccttcattcgggacagcggtatgcagctgatgacgctcaaggcggatggcgacatttccgtgaaggaactcggggacaatccggatcggctggccttgctgttcggcagcgaaaagggtgggccttccgacctgttcgaggaggcgtcttccgcctcggtttccatccccatgatgagccagaccgagtctctcaacgtttccgtttccctcggaatcgcgctgcacgagaggatcgacaggaatctcgcggccaaccgataa

SEQ ID NO: 17 - DNA, 41 bp, synthetic construct
  source 1..41: mol_type = other DNA
  misc_feature 1..41: note = tsr-kpnF
gccggtaccgctagatctccaatatgcggggatcgaccgcg

SEQ ID NO: 18 - DNA, 48 bp, synthetic construct
  source 1..48: mol_type = other DNA
  misc_feature 1..48: note = tsr-xbaR
agcttgggctgcaggtcgactctagattatcggttggccgcgagattc

SEQ ID NO: 19 - DNA, 7560 bp, synthetic construct
  source 1..7560: mol_type = other DNA
  misc_feature 1..7560: note = pSET152-PtipA-gfpuv-tsr
caggcttcccgggtgtctcgctacgccgctacgtcttccgtgccgtcctgggcgtcgtcttcgtcgtcgtcggtcggcggcttcgcccacgtgatcgaagcgcgcttctcgatgggcgttccctgccccctgcccgtagtcgacttcgtgacaacgatcttgtctacgaagagcccgacgaacacgcgcttgtcgtctactgacgcgcgcccccaccacgacttagggccggtcgggtcagcgtcggcgtcttcggggaaccattggtcaaggggaagcttcggggcttcggcggcttcaagttcggcaagccgctcttccgccccttgctgccggagcgtcagcgctgcctgttgcttccggaagtgcttcctgccaacgggtccgtcgtacgcgcctgccgcgcggtcttcgtacagctcttcaagggcgttcagggcgtcggcgcgctccgcaacaaggttcgcccgttcgccgctcttctcaggcgcctcagtgagcttgccgaagcgtcgggcggcttcccacagaagcgccaacgtctcttcgtcgccttcggcgtgcctgatcttgttgaagatgcgttccgcaacgaacttgtcgagtgccgccatgctgacgttgcacgtgccttcgtgctgcccaggtgcggacgggtcgaccaccttccggcgacggcagcggtaagagtccttgatcgattcttccccgcgcttcgaagtcatgacggcgccacactcgcagtacagcttgtccatggcggacagaatggcttgcccccgggaaagccccttgccgcgccccctgccgtccaaccacgcctgaagctcataccactcagcgggctcgatgatcggtccgcaatcaagctcgaccggccggagcgtgatcgggtcgcgctgaatgcggtaaccctcaatcttcgtggtcggcgtgccgtccggcttcttcttgtagatcacctcagcggcgaagcccgcaatacgcgggtcccgaaggattcgcataacggttgccgggtcccaggcgcttgaagcggtcttcttcccaatcgtctcgccccgggtcggcacggcgtcagcgtccatgcgcttacaaagccccgtgatgctgcccgggtgaatggcggcttgactgcccggcttgaagggaaggtgtttgtgcgtcttgatctcacgccaccaccaccggattacgtcgggctcgaactcgaagggtccggtaaggggagtggtcgagtgcgcaagcttgttgatgacgacattgaccattcggccgttgcgcgtgatctccttcgtctccgaaacaagctcgaagccgtaaggcgccttcccgccgacgtacccgcccaattcgcgctgaaggttcttcgtgtcgagaatcttcgccgacttcagcgaagattctttgtgcgacgcgtcgagccgcataatcaggtgaatcaggtccatgacgtttccctgccggaagacgccttcctgagtggaaacaatcgtcacgcccagggcgagcaattccgagacaatcggaatcgcgtccatgaccttcaggcgcgagaagcgcgacacgtcatagacaatgatcatgttgagccgcccggcgcggcattcgttcaggatgcgttcgaactccgggcgctccgccgtcccgaacgccgacgtgcccggcgcttcgctgaaatgcccgacgaacctgaaccggcccccgtcgcgctcgacttcgcgctgaaggtcggccgccttgtcttcgttggcgctacgctgtgtcgctgggcttgctgcgctcgaattctcgcgctcgcgcgactgacggtcgtaagcacccgcgtacgtgtccaccccggtcacaaccccttgtgtcatgtcggcgaccctacgcccccaactgagagaactcaaaggttaccccagttggggcactactcccgaaaaccgcttctgacctgggaaaacgtgaagccccggggcatccgctgagggttgccgccggggcttcggtgtgtccgtcagtacgggccatagaggggcgtcgtgtaacccacccagggcgattgctccggcacggggaagccgcgccacgccttcgggacgtctggaatcgctagagcttgcatgcctgcaggtcgacggatcttttccgctgcataaccctgcttcggggtcattatagcgattttttcggtatatccatcctttttcgcacgatatacaggattttgccaaagggttcgtgtagactttccttggtgtatccaacggcgtcagccgggcaggataggtgaagtaggcccacccgcgagcgggtgttccttcttcactgtcccttattcgcacctggcggtgctcaacgggaatcctgctctgcgaggctggccggctaccgccggcgtaacagatgagggcaagcggatggctgatgaaaccaagccaaccaggaagggcagcccacctatcaaggtgtactgccttccagacgaacgaagagcgattgaggaaaaggcggcggcggccggcatgagcctgtcggcctacctgctggccgtcggccagggctacaaaatcacgggcgtcgtggactatgagcacgtccgcgagctggcccgcatcaatggcgacctgggccgcctgggcggcctgctgaaactctggctcaccgacgacccgcgcacggcgcggttcggtgatgccacgatcctcgccctgctggcgaagatcgaagagaagcaggacgagcttggcaaggtcatgatgggcgtggtccgcccgagggcagagccatgacttttttagccgctaaaacggccggggggtgcgcgtgattgccaagcacgtccccatgcgctccatcaagaagagcgacttcgcggagctggtgaagtacatcaccgacgagcaaggcaagaccgatccccggggacctgcaggtcgactctagctagctggccagggcccgatacgtcgcggtgagttcaggctttttcatatctcattgcccccggacgagcgtctgctccgccattcgccgtccgccgtgccaatcggatcagccgtccaaatgcgggattttcgttagtcggaggccaaacggcattgagcgtcagcatatcatcagcgagctgaagaaagacaatccccgatccgctccacgtgttgccccagcaatcagcgcgaccttgcccctccaacgtcatctcgttctccgctcatgagctcagccaatcgactggcgagcggcatcgcattcttcgcatcccgcctctggcggatgcaggaagatcaacggatctcggcccagttgacccagggctgtcgccacaatgtcgcgggagcggatcaaccgagcaaaggcatgaccgactggaccttccttctgaaggctcttctccttgagccacctgtccgccaaggcaaagcgctcacagcagtggtcattctcgagataatcgacgcgtaccaacttgccatcctgaagaatggtgcagtgtctcggcaccccatagggaacctttgccatcaactcggcaagatgcagcgtcgtgttggcatcgtgtcccacgccgaggagaagtacctgcccatcgagttcatggacacgggcgaccgggcttgcaggcgagtgaggtggcaggggcaatggatcagagatgatctgctctgcctgtggccccgctgccgcaaaggcaaatggatgggcgctgcgctttacatttggcaggcgccagaatgtgtcagagacaactccaaggtccggtgtaacgggcgacgtggcaggatcgaacggctcgtcgtccagacctgaccacgagggcatgacgagcgtccctcccggacccagcgcagcacgcagggcctcgatcagtccaagtggcccatcttcgaggggccggacgctacggaaggagctgtggaccagcagcacaccgccgggggtaaccccaaggttgagaagctgaccgatgagctcggcttttcgccattcgtattgcacgacattgcactccaccgctgatgacatcagtcgatcatagcacgatcaacggcactgttgcaaatagtcggtggtgataaacttatcatccccttttgctgatggagctgcacatgaaccaaaaggatctaggtgaagatcctttttgataatctcatgaccaaaatcccttaacgtgagttttcgttccactgagcgtcagaccccgtagaaaagatcaaaggatcttcttgagatcctttttttctgcgcgtaatctgctgcttgcaaacaaaaaaaccaccgctaccagcggtggtttgtttgccggatcaagagctaccaactctttttccgaaggtaactggcttcagcagagcgcagataccaaatactgttcttctagtgtagccgtagttaggccaccacttcaagaactctgtagcaccgcctacatacctcgctctgctaatcctgttaccagtggctgctgccagtggcgataagtcgtgtcttaccgggttggactcaagacgatagttaccggataaggcgcagcggtcgggctgaacggggggttcgtgcacacagcccagcttggagcgaacgacctacaccgaactgagatacctacagcgtgagctatgagaaagcgccacgcttcccgaagggagaaaggcggacaggtatccggtaagcggcagggtcggaacaggagagcgcacgagggagcttccagggggaaacgcctggtatctttatagtcctgtcgggtttcgccacctctgacttgagcgtcgatttttgtgatgctcgtcaggggggcggagcctatggaaaaacgccagcaacgcggcctttttacggttcctggccttttgctggccttttgctcacatgttctttcctgcgttatcccctgattctgtggataaccgtattaccgcctttgagtgagctgataccgctcgccgcagccgaacgaccgagcgcagcgagtcagtgagcgaggaagcggaagagcgcccaatacgcaaaccgcctctccccgcgcgttggccgattcattaatgcagctggcacgacaggtttcccgactggaaagcgggcagtgagcgcaacgcaattaatgtgagttagctcactcattaggcaccccaggctttacactttatgcttccggctcgtatgttgtgtggaattgtgagcggataacaatttcacacaggaaacagctatgacatgattacgaattcgatatcagggctacgctggaccggatgggctgagggagccgacggcacgcggcggctcacggcgtggcacgcggaacgtccgggcttgcacctcacgtcacgtgaggaggcagcgtggacggcgtcagagaagggagcggagcatatgagcaagggcgaggagctgttcaccggcgtggtgccgatcctggtcgaactggacggggacgtcaacggccacaagttctcggtgtccggtgagggcgaaggcgacgccacgtacggcaagctcaccctgaagttcatctgcacgacgggcaagctgcccgtgccctggcccacgctcgtcacgaccttcagctacggcgtccagtgcttctcgcgctacccggaccacatgaagcggcacgacttcttcaagtccgccatgccggagggctacgtccaggaacgcaccatctccttcaaggacgacggcaactacaagacccgcgcggaggtcaagttcgagggcgacaccctggtcaaccgcatcgagctgaagggcatcgacttcaaggaggacggcaacatcctgggccacaagctcgagtacaactacaactcccacaacgtctacatcaccgccgacaagcagaagaacgggatcaaggcgaacttcaagatccggcacaacatcgaggacggctccgtgcagctggccgaccactaccagcagaacaccccgatcggcgacggtccggtcctgctgcccgacaaccactacctctccacccagtcggccctgtcgaaggacccgaacgagaagcgcgaccacatggtcctcctggagttcgtgaccgcggccgggatcacccacgggatggacgagctctacaagtgagccggtaccgctagatctccaatatgcggggatcgaccgcgcgggtcccggacggggaagagcggggagctttgccagagagcgacgacttccccttgcgttggtgattgccggtcagggcagccatccgccatcgtcgcgtagggtgtcacaccccaggaatcgcgtcactgaacacagcagccggtaggacgaccatgactgagttggacaccatcgcaaatccgtccgatcccgcggtgcagcggatcatcgatgtcaccaagccgtcgcgatccaacataaagacaacgttgatcgaggacgtcgagcccctcatgcacagcatcgcggccggggtggagttcatcgaggtctacggcagcgacagcagtccttttccatctgagttgctggatctgtgcgggcggcagaacataccggtccgcctcatcgactcctcgatcgtcaaccagttgttcaagggggagcggaaggccaagacattcggcatcgcccgcgtccctcgcccggccaggttcggcgatatcgcgagccggcgtggggacgtcgtcgttctcgacggggtgaagatcgtcgggaacatcggcgcgatagtacgcacgtcgctcgcgctcggagcgtcggggatcatcctggtcgacagtgacatcaccagcatcgcggaccggcgtctccaaagggccagccgaggttacgtcttctcccttcccgtcgttctctccggtcgcgaggaggccatcgccttcattcgggacagcggtatgcagctgatgacgctcaaggcggatggcgacatttccgtgaaggaactcggggacaatccggatcggctggccttgctgttcggcagcgaaaagggtgggccttccgacctgttcgaggaggcgtcttccgcctcggtttccatccccatgatgagccagaccgagtctctcaacgtttccgtttccctcggaatcgcgctgcacgagaggatcgacaggaatctcgcggccaaccgataatctagagtcgacctgcagcccaagcttggcactggccgtcgttttacaacgtcgtgactgggaaaaccctggcgttacccaacttaatcgccttgcagcacatccccctttcgccagctggcgtaatagcgaagaggcccgcaccgatcgcccttcccaacagttgcgcagcctgaatggcgaatggcgcctgatgcggtattttctccttacgcatctgtgcggtatttcacaccgcataaattccccaatgtcaagcacttccggaatcgggagcgcggccgatgcaaagtgccgatcaacataacgatctttgtagaaaccatcggcgcagctatttacccgcaggacatatccacgccctcctacatcgaagctgaaagcacgagattcttcgccctgcgagagctgcatcaggtcggagacgctgtcgaacttttcgatcagaaacttctcgacagacgtagat

SEQ ID NO: 20 - DNA, 2124 bp, synthetic construct
  source 1..2124: mol_type = other DNA
  misc_feature 1..2124: note = pSG5 ori (synthetic)
gactagtcaagcttcggatcctgcccgccgaacgcgtcgtcgtcgacggcctggtgctcatcgacgagcacccggagccaggtgaaaagcgccggcggacgctcggactgggcgcgggattccagcagtaacccaggtccgccggccacctcacggcaggcagaccctcggctttcgcgccgggaccgccatgagaccgccacccggatgtccggggtggcggtctcatggcggtccctcagcggccctacgcgaccgctgtgtcgacgcggaggcagtctccggggagccggccccagggctggagtaccggggcgagcttgcccttgcagcggcggcacacgggcgacgcggcgccgggcgggggagtcttgacgtcgacggtgaccggcttcggcttcaggcgcttccgaaggctgatcgtcgggcggatcgcctccttcttcggctgacgcactcggtcgagcgaagcggccagctcctccgtgcgggcctcgttggccttccggcgcgcctcgcggaaagcagcttcctcctcggacatgacctcgaacctcatctggtcagcgtcaaggtcgcccggcgcggccggcgcttccggggcgggcgggtccaggacgtccttgccccacaccaggccccaggactcgacgagccgccggacgcccggtaggccgtacgtctcggcgaccttgatgaggtcgaggcgacgtccggcgacgcgggcgatgtatcggtaccagatgtaggccgggatgaccgcgatggcgaccaggccctcggtgtcgtcggtgatctcctcctcggtgcggacgtcctgctggatgccgagttccttgatcagccggttcaggttctgcgaccggtagtgcttgcggacctggaagacgccgaactcgcgctcgcggtacttctcgacgaacgggccgggccgacgaagccgctgcagctcggcggccgccgcgtcgcccaggtcgagcggtcccatgcggtcgtcgccgcgaccggccttgaagttctgtccggccagctccaggccgatcttggcgacgccgcccttggtcttgtcgccgtccttgtagaggtagcgggcctgcttgcccgcatcgccgtcagcggcgtccgcgccgttgagtgggcgcacgtcggtgccgtggcccttgccctcacaggagcaaccgggccggtcgcacgtctcgctgacggtgtagccgcccgcggattcgaccccggcggcccaggctccggcgagtgcgtcgcggaacgcggcctgggcgtccgggccgagcacctcgcgggtgacccagagcgtgtgccagtgcaggtgccagccggagccccagccgaaggtgtcctcgaaggcccgctcgtagccgatgatcccgaagtcgtcgcgcatcgtgcgccagcggcggccggacgagccgtacgcgcccttccagccgtcgtgcaagaccgcgaccaggccgtgccgcattcccttgcggacggtgccgaacgccatgcgctcgaagtggcgcaacgtgttcgtgccaaggtgcagcccgtacccggcgtccgcgagaccgtcggcggcgagctgcacgttcgagccccgtacggccaggatgcggctcatgcaccacgggcaggtgtggacgttgttgcagcggcacgtgttgccccacgtcgcctcgcccggcttccacatcagctcggccgtcccggcagtgagccgggtcccgcagcccttgaacgcctcgttcagcgacaccgtctggtgccggtcccgccgggcgaaccgctcgtcgcgcgggtcctcccgcccggctgtcgcggcaccctcgtttggggtagaacccgttccagttacagcgctctgacctgcagtggacggagattttcccttactactaaagcccgcgtccggattacccgctgtagtcgtgcttgctacgctgcgtgactggtccgcaatgagacgctttgcgcgctttcggcaggcgtccgagcagtagattttggggcgcttcccggggatgtggacgatcggggtgccgcagtggcacttcggtccggcggggcgcggtggtgtcgacgcgctgttctctcgtacgctcgtcacagagcaaacgtcctcactcg

SEQ ID NO: 21 - DNA, 7109 bp, synthetic construct
  source 1..7109: mol_type = other DNA
  misc_feature 1..7109: note = pSET152-PtipA-gfpuv-pSG5rep
aagatcaaaggatcttcttgagatcctttttttctgcgcgtaatctgctgcttgcaaacaaaaaaaccaccgctaccagcggtggtttgtttgccggatcaagagctaccaactctttttccgaaggtaactggcttcagcagagcgcagataccaaatactgttcttctagtgtagccgtagttaggccaccacttcaagaactctgtagcaccgcctacatacctcgctctgctaatcctgttaccagtggctgctgccagtggcgataagtcgtgtcttaccgggttggactcaagacgatagttaccggataaggcgcagcggtcgggctgaacggggggttcgtgcacacagcccagcttggagcgaacgacctacaccgaactgagatacctacagcgtgagctatgagaaagcgccacgcttcccgaagggagaaaggcggacaggtatccggtaagcggcagggtcggaacaggagagcgcacgagggagcttccagggggaaacgcctggtatctttatagtcctgtcgggtttcgccacctctgacttgagcgtcgatttttgtgatgctcgtcaggggggcggagcctatggaaaaacgccagcaacgcggcctttttacggttcctggccttttgctggccttttgctcacatgttctttcctgcgttatcccctgattctgtggataaccgtattaccgcctttgagtgagctgataccgctcgccgcagccgaacgaccgagcgcagcgagtcagtgagcgaggaagcggaagagcgcccaatacgcaaaccgcctctccccgcgcgttggccgattcattaatgcagctggcacgacaggtttcccgactggaaagcgggcagtgagcgcaacgcaattaatgtgagttagctcactcattaggcaccccaggctttacactttatgcttccggctcgtatgttgtgtggaattgtgagcggataacaatttcacacaggaaacagctatgacatgattacgaattcgatatcagggctacgctggaccggatgggctgagggagccgacggcacgcggcggctcacggcgtggcacgcggaacgtccgggcttgcacctcacgtcacgtgaggaggcagcgtggacggcgtcagagaagggagcggagcatagcaagggcgaggagctgttcaccggcgtggtgccgatcctggtcgaactggacggggacgtcaacggccacaagttctcggtgtccggtgagggcgaaggcgacgccacgtacggcaagctcaccctgaagttcatctgcacgacgggcaagctgcccgtgccctggcccacgctcgtcacgaccttcagctacggcgtccagtgcttctcgcgctacccggaccacatgaagcggcacgacttcttcaagtccgccatgccggagggctacgtccaggaacgcaccatctccttcaaggacgacggcaactacaagacccgcgcggaggtcaagttcgagggcgacaccctggtcaaccgcatcgagctgaagggcatcgacttcaaggaggacggcaacatcctgggccacaagctcgagtacaactacaactcccacaacgtctacatcaccgccgacaagcagaagaacgggatcaaggcgaacttcaagatccggcacaacatcgaggacggctccgtgcagctggccgaccactaccagcagaacaccccgatcggcgacggtccggtcctgctgcccgacaaccactacctctccacccagtcggccctgtcgaaggacccgaacgagaagcgcgaccacatggtcctcctggagttcgtgaccgcggccgggatcacccacgggatggacgagctctacaagtgagccggtaccgctagatctccaatatgcggggatcgaccgcgcgggtcccggacggggaagagcggggagctttgccagagagcgacgacttccccttgcgttggtgattgccggtcagggcagccatccgccatcgtcgcgtagggtgtcacaccccaggaatcgcgtcactgaacacagcagccggtaggacgaccatgactgagttggacaccatcgcaaatccgtccgatcccgcggtgcagcggatcatcgatgtcaccaagccgtcgcgatccaacataaagacaacgttgatcgaggacgtcgagcccctcatgcacagcatcgcggccggggtggagttcatcgaggtctacggcagcgacagcagtccttttccatctgagttgctggatctgtgcgggcggcagaacataccggtccgcctcatcgactcctcgatcgtcaaccagttgttcaagggggagcggaaggccaagacattcggcatcgcccgcgtccctcgcccggccaggttcggcgatatcgcgagccggcgtggggacgtcgtcgttctcgacggggtgaagatcgtcgggaacatcggcgcgatagtacgcacgtcgctcgcgctcggagcgtcggggatcatcctggtcgacagtgacatcaccagcatcgcggaccggcgtctccaaagggccagccgaggttacgtcttctcccttcccgtcgttctctccggtcgcgaggaggccatcgccttcattcgggacagcggtatgcagctgatgacgctcaaggcggatggcgacatttccgtgaaggaactcggggacaatccggatcggctggccttgctgttcggcagcgaaaagggtgggccttccgacctgttcgaggaggcgtcttccgcctcggtttccatccccatgatgagccagaccgagtctctcaacgtttccgtttccctcggaatcgcgctgcacgagaggatcgacaggaatctcgcggccaaccgataatctagagactagtcaagcttcggatcctgcccgccgaacgcgtcgtcgtcgacggcctggtgctcatcgacgagcacccggagccaggtgaaaagcgccggcggacgctcggactgggcgcgggattccagcagtaacccaggtccgccggccacctcacggcaggcagaccctcggctttcgcgccgggaccgccatgagaccgccacccggatgtccggggtggcggtctcatggcggtccctcagcggccctacgcgaccgctgtgtcgacgcggaggcagtctccggggagccggccccagggctggagtaccggggcgagcttgcccttgcagcggcggcacacgggcgacgcggcgccgggcgggggagtcttgacgtcgacggtgaccggcttcggcttcaggcgcttccgaaggctgatcgtcgggcggatcgcctccttcttcggctgacgcactcggtcgagcgaagcggccagctcctccgtgcgggcctcgttggccttccggcgcgcctcgcggaaagcagcttcctcctcggacatgacctcgaacctcatctggtcagcgtcaaggtcgcccggcgcggccggcgcttccggggcgggcgggtccaggacgtccttgccccacaccaggccccaggactcgacgagccgccggacgcccggtaggccgtacgtctcggcgaccttgatgaggtcgaggcgacgtccggcgacgcgggcgatgtatcggtaccagatgtaggccgggatgaccgcgatggcgaccaggccctcggtgtcgtcggtgatctcctcctcggtgcggacgtcctgctggatgccgagttccttgatcagccggttcaggttctgcgaccggtagtgcttgcggacctggaagacgccgaactcgcgctcgcggtacttctcgacgaacgggccgggccgacgaagccgctgcagctcggcggccgccgcgtcgcccaggtcgagcggtcccatgcggtcgtcgccgcgaccggccttgaagttctgtccggccagctccaggccgatcttggcgacgccgcccttggtcttgtcgccgtccttgtagaggtagcgggcctgcttgcccgcatcgccgtcagcggcgtccgcgccgttgagtgggcgcacgtcggtgccgtggcccttgccctcacaggagcaaccgggccggtcgcacgtctcgctgacggtgtagccgcccgcggattcgaccccggcggcccaggctccggcgagtgcgtcgcggaacgcggcctgggcgtccgggccgagcacctcgcgggtgacccagagcgtgtgccagtgcaggtgccagccggagccccagccgaaggtgtcctcgaaggcccgctcgtagccgatgatcccgaagtcgtcgcgcatcgtgcgccagcggcggccggacgagccgtacgcgcccttccagccgtcgtgcaagaccgcgaccaggccgtgccgcattcccttgcggacggtgccgaacgccatgcgctcgaagtggcgcaacgtgttcgtgccaaggtgcagcccgtacccggcgtccgcgagaccgtcggcggcgagctgcacgttcgagccccgtacggccaggatgcggctcatgcaccacgggcaggtgtggacgttgttgcagcggcacgtgttgccccacgtcgcctcgcccggcttccacatcagctcggccgtcccggcagtgagccgggtcccgcagcccttgaacgcctcgttcagcgacaccgtctggtgccggtcccgccgggcgaaccgctcgtcgcgcgggtcctcccgcccggctgtcgcggcaccctcgtttggggtagaacccgttccagttacagcgctctgacctgcagtggacggagattttcccttactactaaagcccgcgtccggattacccgctgtagtcgtgcttgctacgctgcgtgactggtccgcaatgagacgctttgcgcgctttcggcaggcgtccgagcagtagattttggggcgcttcccggggatgtggacgatcggggtgccgcagtggcacttcggtccggcggggcgcggtggtgtcgacgcgctgttctctcgtacgctcgtcacagagcaaacgtcctcactcggcatgcctgcaggtcgacggatcttttccgctgcataaccctgcttcggggtcattatagcgattttttcggtatatccatcctttttcgcacgatatacaggattttgccaaagggttcgtgtagactttccttggtgtatccaacggcgtcagccgggcaggataggtgaagtaggcccacccgcgagcgggtgttccttcttcactgtcccttattcgcacctggcggtgctcaacgggaatcctgctctgcgaggctggccggctaccgccggcgtaacagatgagggcaagcggatggctgatgaaaccaagccaaccaggaagggcagcccacctatcaaggtgtactgccttccagacgaacgaagagcgattgaggaaaaggcggcggcggccggcatgagcctgtcggcctacctgctggccgtcggccagggctacaaaatcacgggcgtcgtggactatgagcacgtccgcgagctggcccgcatcaatggcgacctgggccgcctgggcggcctgctgaaactctggctcaccgacgacccgcgcacggcgcggttcggtgatgccacgatcctcgccctgctggcgaagatcgaagagaagcaggacgagcttggcaaggtcatgatgggcgtggtccgcccgagggcagagccatgacttttttagccgctaaaacggccggggggtgcgcgtgattgccaagcacgtccccatgcgctccatcaagaagagcgacttcgcggagctggtgaagtacatcaccgacgagcaaggcaagaccgatccccggggacctgcaggtcgactctagctagctggccagggcccgatacgtcgcggtgagttcaggctttttcatatctcattgcccccggacgagcgtctgctccgccattcgccgtccgccgtgccaatcggatcagccgtccaaatgcgggattttcgttagtcggaggccaaacggcattgagcgtcagcatatcatcagcgagctgaagaaagacaatccccgatccgctccacgtgttgccccagcaatcagcgcgaccttgcccctccaacgtcatctcgttctccgctcatgagctcagccaatcgactggcgagcggcatcgcattcttcgcatcccgcctctggcggatgcaggaagatcaacggatctcggcccagttgacccagggctgtcgccacaatgtcgcgggagcggatcaaccgagcaaaggcatgaccgactggaccttccttctgaaggctcttctccttgagccacctgtccgccaaggcaaagcgctcacagcagtggtcattctcgagataatcgacgcgtaccaacttgccatcctgaagaatggtgcagtgtctcggcaccccatagggaacctttgccatcaactcggcaagatgcagcgtcgtgttggcatcgtgtcccacgccgaggagaagtacctgcccatcgagttcatggacacgggcgaccgggcttgcaggcgagtgaggtggcaggggcaatggatcagagatgatctgctctgcctgtggccccgctgccgcaaaggcaaatggatgggcgctgcgctttacatttggcaggcgccagaatgtgtcagagacaactccaaggtccggtgtaacgggcgacgtggcaggatcgaacggctcgtcgtccagacctgaccacgagggcatgacgagcgtccctcccggacccagcgcagcacgcagggcctcgatcagtccaagtggcccatcttcgaggggccggacgctacggaaggagctgtggaccagcagcacaccgccgggggtaaccccaaggttgagaagctgaccgatgagctcggcttttcgccattcgtattgcacgacattgcactccaccgctgatgacatcagtcgatcatagcacgatcaacggcactgttgcaaatagtcggtggtgataaacttatcatccccttttgctgatggagctgcacatgaaccaaaaggatctaggtgaagatcctttttgataatctcatgaccaaaatcccttaacgtgagttttcgttccactgagcgtcagaccccgtagaa

SEQ ID NO: 22 - DNA, 429 bp, synthetic construct
  source 1..429: mol_type = other DNA
  misc_feature 1..429: note = pacI (codon optimized)
atgacgcagtgcccgcgctgccagcggaacctcgcggccgacgagttctacgccgggtcctccaagatgtgcaaggggtgcatgacgtggcagaacctcagctacaacgcgaacaaggaaggccacgcgaacacgttcaccaaggccaccttcctggcctggtacgggctgtccgcgcagcggcactgcgggtactgcgggatctccgaagcggggttcacctccctccaccggacgaacccgcgggggtaccacatccagtgcctgggcgtggaccgctccgacagcttcgagggctactccccccagaacgcccgcctcgcctgcttcatctgcaaccggatcaagagcaacatcttctcggcgtccgagatggacgtgctcggggaggccatctcgaaggcgtggcacgggcgggggatcgcctag

SEQ ID NO: 23 - DNA, 31 bp, synthetic construct
  source 1..31: mol_type = other DNA
  misc_feature 1..31: note = pacI-ndeF
agcggacgcatatgacgcagtgcccgcgctg

SEQ ID NO: 24 - DNA, 32 bp, synthetic construct
  source 1..32: mol_type = other DNA
  misc_feature 1..32: note = pacI-bglR
tgcacatgaacctaggcgatcccccgcccgtg

SEQ ID NO: 25 - DNA, 1267 bp, synthetic construct
  source 1..1267: mol_type = other DNA
  misc_feature 1..1267: note = lacI
ctactgggctgcttcctaatgcaggagtcgcataagggagagcgtcgagatcccggacaccatcgaatggcgcaaaacctttcgcggtatggcatgatagcgcccggaagagagtcaattcagggtggtgaatgtgaaaccagtaacgttatacgatgtcgcagagtatgccggtgtctcttatcagaccgtttcccgcgtggtgaaccaggccagccacgtttctgcgaaaacgcgggaaaaagtggaagcggcgatggcggagctgaattacattcccaaccgcgtggcacaacaactggcgggcaaacagtcgttgctgattggcgttgccacctccagtctggccctgcacgcgccgtcgcaaattgtcgcggcgattaaatctcgcgccgatcaactgggtgccagcgtggtggtgtcgatggtagaacgaagcggcgtcgaagcctgtaaagcggcggtgcacaatcttctcgcgcaacgcgtcagtgggctgatcattaactatccgctggatgaccaggatgccattgctgtggaagctgcctgcactaatgttccggcgttatttcttgatgtctctgaccagacacccatcaacagtattattttctcccatgaagacggtacgcgactgggcgtggagcatctggtcgcattgggtcaccagcaaatcgcgctgttagcgggcccattaagttctgtctcggcgcgtctgcgtctggctggctggcataaatatctcactcgcaatcaaattcagccgatagcggaacgggaaggcgactggagtgccatgtccggttttcaacaaaccatgcaaatgctgaatgagggcatcgttcccactgcgatgctggttgccaacgatcagatggcgctgggcgcaatgcgcgccattaccgagtccgggctgcgcgttggtgcggatatctcggtagtgggatacgacgataccgaagacagctcatgttatatcccgccgttaaccaccatcaaacaggattttcgcctgctggggcaaaccagcgtggaccgcttgctgcaactctctcagggccaggcggtgaagggcaatcagctgttgcccgtctcactggtgaaaagaaaaaccaccctggcgcccaatacgcaaaccgcctctccccgcgcgttggccgattcattaatgcagctggcacgacaggtttcccgactggaaagcgggcagtgagcgcaacgcaattaatgtaagttagctcactcattaggcaccgggatctcg

SEQ ID NO: 26 - DNA, 25 bp, synthetic construct
  source 1..25: mol_type = other DNA
  misc_feature 1..25: note = lacO
ggaattgtgagcggataacaattcc

SEQ ID NO: 27 - DNA, 140 bp, synthetic construct
  source 1..140: mol_type = other DNA
  misc_feature 1..140: note = PtipA(lacO )
gggctgagggagccgacggcacgcggcggctcacggcgtggcacgcggaacgtccgggcttgcacctcacgtcacgtgaggaggcagcgtggacggaattgtgagcggataacaattccggcgtcagagaagggagcgga

SEQ ID NO: 28 - DNA, 54 bp, synthetic construct; identical to SEQ ID NO: 8
  source 1..54: mol_type = other DNA
  misc_feature 1..54: note = tipA-1F

SEQ ID NO: 29 - DNA, 42 bp, synthetic construct
  source 1..42: mol_type = other DNA
  misc_feature 1..42: note = tipA-(lacO)-R
attgttatccgctcacaattccacgctgcctcctcacgtgac

SEQ ID NO: 30 - DNA, 44 bp, synthetic construct
  source 1..44: mol_type = other DNA
  misc_feature 1..44: note = gfpuv-(lacO)-F
aattgtgagcggataacaattccggacggcgtcagagaagggag

SEQ ID NO: 31 - DNA, 44 bp, synthetic construct; identical to SEQ ID NO: 14
  source 1..44: mol_type = other DNA
  misc_feature 1..44: note = gfpuv-MCS-R

SEQ ID NO: 32 - DNA, 41 bp, synthetic construct; identical to SEQ ID NO: 17
  source 1..41: mol_type = other DNA
  misc_feature 1..41: note = tsr-MCS-F

SEQ ID NO: 33 - DNA, 48 bp, synthetic construct; identical to SEQ ID NO: 18
  source 1..48: mol_type = other DNA
  misc_feature 1..48: note = tsr-XbaI-R

SEQ ID NO: 34 - DNA, 7143 bp, synthetic construct
  source 1..7143: mol_type = other DNA
  misc_feature 1..7143: note = pSET152-PtipA(lacO)-gfpuv-pSG5rep
cgggcttgcaggcgagtgaggtggcaggggcaatggatcagagatgatctgctctgcctgtggccccgctgccgcaaaggcaaatggatgggcgctgcgctttacatttggcaggcgccagaatgtgtcagagacaactccaaggtccggtgtaacgggcgacgtggcaggatcgaacggctcgtcgtccagacctgaccacgagggcatgacgagcgtccctcccggacccagcgcagcacgcagggcctcgatcagtccaagtggcccatcttcgaggggccggacgctacggaaggagctgtggaccagcagcacaccgccgggggtaaccccaaggttgagaagctgaccgatgagctcggcttttcgccattcgtattgcacgacattgcactccaccgctgatgacatcagtcgatcatagcacgatcaacggcactgttgcaaatagtcggtggtgataaacttatcatccccttttgctgatggagctgcacatgaaccaaaaggatctaggtgaagatcctttttgataatctcatgaccaaaatcccttaacgtgagttttcgttccactgagcgtcagaccccgtagaaaagatcaaaggatcttcttgagatcctttttttctgcgcgtaatctgctgcttgcaaacaaaaaaaccaccgctaccagcggtggtttgtttgccggatcaagagctaccaactctttttccgaaggtaactggcttcagcagagcgcagataccaaatactgttcttctagtgtagccgtagttaggccaccacttcaagaactctgtagcaccgcctacatacctcgctctgctaatcctgttaccagtggctgctgccagtggcgataagtcgtgtcttaccgggttggactcaagacgatagttaccggataaggcgcagcggtcgggctgaacggggggttcgtgcacacagcccagcttggagcgaacgacctacaccgaactgagatacctacagcgtgagctatgagaaagcgccacgcttcccgaagggagaaaggcggacaggtatccggtaagcggcagggtcggaacaggagagcgcacgagggagcttccagggggaaacgcctggtatctttatagtcctgtcgggtttcgccacctctgacttgagcgtcgatttttgtgatgctcgtcaggggggcggagcctatggaaaaacgccagcaacgcggcctttttacggttcctggccttttgctggccttttgctcacatgttctttcctgcgttatcccctgattctgtggataaccgtattaccgcctttgagtgagctgataccgctcgccgcagccgaacgaccgagcgcagcgagtcagtgagcgaggaagcggaagagcgcccaatacgcaaaccgcctctccccgcgcgttggccgattcattaatgcagctggcacgacaggtttcccgactggaaagcgggcagtgagcgcaacgcaattaatgtgagttagctcactcattaggcaccccaggctttacactttatgcttccggctcgtatgttgtgtggaattgtgagcggataacaatttcacacaggaaacagctatgacatgattacgaattcgatatcagggctacgctggaccggatgggctgagggagccgacggcacgcggcggctcacggcgtggcacgcggaacgtccgggcttgcacctcacgtcacgtgaggaggcagcgtggacggccatggggaattgtgagcggataacaattcccgtcagagaagggagcggagcatatgagcaagggcgaggagctgttcaccggcgtggtgccgatcctggtcgaactggacggggacgtcaacggccacaagttctcggtgtccggtgagggcgaaggcgacgccacgtacggcaagctcaccctgaagttcatctgcacgacgggcaagctgcccgtgccctggcccacgctcgtcacgaccttcagctacggcgtccagtgcttctcgcgctacccggaccacatgaagcggcacgacttcttcaagtccgccatgccggagggctacgtccaggaacgcaccatctccttcaaggacgacggcaactacaagacccgcgcggaggtcaagttcgagggcgacaccctggtcaaccgcatcgagctgaagggcatcgacttcaaggaggacggcaacatcctgggccacaagctcgagtacaactacaactcccacaacgtctacatcaccgccgacaagcagaagaacgggatcaaggcgaacttcaagatccggcacaacatcgaggacggctccgtgcagctggccgaccactaccagcagaacaccccgatcggcgacggtccggtcctgctgcccgacaaccactacctctccacccagtcggccctgtcgaaggacccgaacgagaagcgcgaccacatggtcctcctggagttcgtgaccgcggccgggatcacccacgggatggacgagctctacaagtgagccggtaccgctagatctccaatatgcggggatcgaccgcgcgggtcccggacggggaagagcggggagctttgccagagagcgacgacttccccttgcgttggtgattgccggtcagggcagccatccgccatcgtcgcgtagggtgtcacaccccaggaatcgcgtcactgaacacagcagccggtaggacgaccatgactgagttggacaccatcgcaaatccgtccgatcccgcggtgcagcggatcatcgatgtcaccaagccgtcgcgatccaacataaagacaacgttgatcgaggacgtcgagcccctcatgcacagcatcgcggccggggtggagttcatcgaggtctacggcagcgacagcagtccttttccatctgagttgctggatctgtgcgggcggcagaacataccggtccgcctcatcgactcctcgatcgtcaaccagttgttcaagggggagcggaaggccaagacattcggcatcgcccgcgtccctcgcccggccaggttcggcgatatcgcgagccggcgtggggacgtcgtcgttctcgacggggtgaagatcgtcgggaacatcggcgcgatagtacgcacgtcgctcgcgctcggagcgtcggggatcatcctggtcgacagtgacatcaccagcatcgcggaccggcgtctccaaagggccagccgaggttacgtcttctcccttcccgtcgttctctccggtcgcgaggaggccatcgccttcattcgggacagcggtatgcagctgatgacgctcaaggcggatggcgacatttccgtgaaggaactcggggacaatccggatcggctggccttgctgttcggcagcgaaaagggtgggccttccgacctgttcgaggaggcgtcttccgcctcggtttccatccccatgatgagccagaccgagtctctcaacgtttccgtttccctcggaatcgcgctgcacgagaggatcgacaggaatctcgcggccaaccgataatctagagactagtcaagcttcggatcctgcccgccgaacgcgtcgtcgtcgacggcctggtgctcatcgacgagcacccggagccaggtgaaaagcgccggcggacgctcggactgggcgcgggattccagcagtaacccaggtccgccggccacctcacggcaggcagaccctcggctttcgcgccgggaccgccatgagaccgccacccggatgtccggggtggcggtctcatggcggtccctcagcggccctacgcgaccgctgtgtcgacgcggaggcagtctccggggagccggccccagggctggagtaccggggcgagcttgcccttgcagcggcggcacacgggcgacgcggcgccgggcgggggagtcttgacgtcgacggtgaccggcttcggcttcaggcgcttccgaaggctgatcgtcgggcggatcgcctccttcttcggctgacgcactcggtcgagcgaagcggccagctcctccgtgcgggcctcgttggccttccggcgcgcctcgcggaaagcagcttcctcctcggacatgacctcgaacctcatctggtcagcgtcaaggtcgcccggcgcggccggcgcttccggggcgggcgggtccaggacgtccttgccccacaccaggccccaggactcgacgagccgccggacgcccggtaggccgtacgtctcggcgaccttgatgaggtcgaggcgacgtccggcgacgcgggcgatgtatcggtaccagatgtaggccgggatgaccgcgatggcgaccaggccctcggtgtcgtcggtgatctcctcctcggtgcggacgtcctgctggatgccgagttccttgatcagccggttcaggttctgcgaccggtagtgcttgcggacctggaagacgccgaactcgcgctcgcggtacttctcgacgaacgggccgggccgacgaagccgctgcagctcggcggccgccgcgtcgcccaggtcgagcggtcccatgcggtcgtcgccgcgaccggccttgaagttctgtccggccagctccaggccgatcttggcgacgccgcccttggtcttgtcgccgtccttgtagaggtagcgggcctgcttgcccgcatcgccgtcagcggcgtccgcgccgttgagtgggcgcacgtcggtgccgtggcccttgccctcacaggagcaaccgggccggtcgcacgtctcgctgacggtgtagccgcccgcggattcgaccccggcggcccaggctccggcgagtgcgtcgcggaacgcggcctgggcgtccgggccgagcacctcgcgggtgacccagagcgtgtgccagtgcaggtgccagccggagccccagccgaaggtgtcctcgaaggcccgctcgtagccgatgatcccgaagtcgtcgcgcatcgtgcgccagcggcggccggacgagccgtacgcgcccttccagccgtcgtgcaagaccgcgaccaggccgtgccgcattcccttgcggacggtgccgaacgccatgcgctcgaagtggcgcaacgtgttcgtgccaaggtgcagcccgtacccggcgtccgcgagaccgtcggcggcgagctgcacgttcgagccccgtacggccaggatgcggctcatgcaccacgggcaggtgtggacgttgttgcagcggcacgtgttgccccacgtcgcctcgcccggcttccacatcagctcggccgtcccggcagtgagccgggtcccgcagcccttgaacgcctcgttcagcgacaccgtctggtgccggtcccgccgggcgaaccgctcgtcgcgcgggtcctcccgcccggctgtcgcggcaccctcgtttggggtagaacccgttccagttacagcgctctgacctgcagtggacggagattttcccttactactaaagcccgcgtccggattacccgctgtagtcgtgcttgctacgctgcgtgactggtccgcaatgagacgctttgcgcgctttcggcaggcgtccgagcagtagattttggggcgcttcccggggatgtggacgatcggggtgccgcagtggcacttcggtccggcggggcgcggtggtgtcgacgcgctgttctctcgtacgctcgtcacagagcaaacgtcctcactcggcatgcctgcaggtcgacggatcttttccgctgcataaccctgcttcggggtcattatagcgattttttcggtatatccatcctttttcgcacgatatacaggattttgccaaagggttcgtgtagactttccttggtgtatccaacggcgtcagccgggcaggataggtgaagtaggcccacccgcgagcgggtgttccttcttcactgtcccttattcgcacctggcggtgctcaacgggaatcctgctctgcgaggctggccggctaccgccggcgtaacagatgagggcaagcggatggctgatgaaaccaagccaaccaggaagggcagcccacctatcaaggtgtactgccttccagacgaacgaagagcgattgaggaaaaggcggcggcggccggcatgagcctgtcggcctacctgctggccgtcggccagggctacaaaatcacgggcgtcgtggactatgagcacgtccgcgagctggcccgcatcaatggcgacctgggccgcctgggcggcctgctgaaactctggctcaccgacgacccgcgcacggcgcggttcggtgatgccacgatcctcgccctgctggcgaagatcgaagagaagcaggacgagcttggcaaggtcatgatgggcgtggtccgcccgagggcagagccatgacttttttagccgctaaaacggccggggggtgcgcgtgattgccaagcacgtccccatgcgctccatcaagaagagcgacttcgcggagctggtgaagtacatcaccgacgagcaaggcaagaccgatccccggggacctgcaggtcgactctagctagctggccagggcccgatacgtcgcggtgagttcaggctttttcatatctcattgcccccggacgagcgtctgctccgccattcgccgtccgccgtgccaatcggatcagccgtccaaatgcgggattttcgttagtcggaggccaaacggcattgagcgtcagcatatcatcagcgagctgaagaaagacaatccccgatccgctccacgtgttgccccagcaatcagcgcgaccttgcccctccaacgtcatctcgttctccgctcatgagctcagccaatcgactggcgagcggcatcgcattcttcgcatcccgcctctggcggatgcaggaagatcaacggatctcggcccagttgacccagggctgtcgccacaatgtcgcgggagcggatcaaccgagcaaaggcatgaccgactggaccttccttctgaaggctcttctccttgagccacctgtccgccaaggcaaagcgctcacagcagtggtcattctcgagataatcgacgcgtaccaacttgccatcctgaagaatggtgcagtgtctcggcaccccatagggaacctttgccatcaactcggcaagatgcagcgtcgtgttggcatcgtgtcccacgccgaggagaagtacctgcccatcgagttcatggacacgggcgac

SEQ ID NO: 35 - DNA, 1267 bp, synthetic construct; identical to SEQ ID NO: 25
  source 1..1267: mol_type = other DNA
  misc_feature 1..1267: note = lacI with its own promoter region (on pET21b)

SEQ ID NO: 36 - DNA, 35 bp, synthetic construct
  source 1..35: mol_type = other DNA
  misc_feature 1..35: note = lacI-NheI-F
gactctagctagcctactgggctgcttcctaatgc

SEQ ID NO: 37 - DNA, 33 bp, synthetic construct
  source 1..33: mol_type = other DNA
  misc_feature 1..33: note = lacI-NheI-R
ctggccagctagccgagatcccggtgcctaatg

SEQ ID NO: 38 - DNA, 8110 bp, synthetic construct
  source 1..8110: mol_type = other DNA
  misc_feature 1..8110: note = pSET152-PtipA(lacO)-pacI-pSG5rep-lacI (pELIM)
gacggatcttttccgctgcataaccctgcttcggggtcattatagcgattttttcggtatatccatcctttttcgcacgatatacaggattttgccaaagggttcgtgtagactttccttggtgtatccaacggcgtcagccgggcaggataggtgaagtaggcccacccgcgagcgggtgttccttcttcactgtcccttattcgcacctggcggtgctcaacgggaatcctgctctgcgaggctggccggctaccgccggcgtaacagatgagggcaagcggatggctgatgaaaccaagccaaccaggaagggcagcccacctatcaaggtgtactgccttccagacgaacgaagagcgattgaggaaaaggcggcggcggccggcatgagcctgtcggcctacctgctggccgtcggccagggctacaaaatcacgggcgtcgtggactatgagcacgtccgcgagctggcccgcatcaatggcgacctgggccgcctgggcggcctgctgaaactctggctcaccgacgacccgcgcacggcgcggttcggtgatgccacgatcctcgccctgctggcgaagatcgaagagaagcaggacgagcttggcaaggtcatgatgggcgtggtccgcccgagggcagagccatgacttttttagccgctaaaacggccggggggtgcgcgtgattgccaagcacgtccccatgcgctccatcaagaagagcgacttcgcggagctggtgaagtacatcaccgacgagcaaggcaagaccgatccccggggacctgcaggtcgactctagctagcctactgggctgcttcctaatgcaggagtcgcataagggagagcgtcgagatcccggacaccatcgaatggcgcaaaacctttcgcggtatggcatgatagcgcccggaagagagtcaattcagggtggtgaatgtgaaaccagtaacgttatacgatgtcgcagagtatgccggtgtctcttatcagaccgtttcccgcgtggtgaaccaggccagccacgtttctgcgaaaacgcgggaaaaagtggaagcggcgatggcggagctgaattacattcccaaccgcgtggcacaacaactggcgggcaaacagtcgttgctgattggcgttgccacctccagtctggccctgcacgcgccgtcgcaaattgtcgcggcgattaaatctcgcgccgatcaactgggtgccagcgtggtggtgtcgatggtagaacgaagcggcgtcgaagcctgtaaagcggcggtgcacaatcttctcgcgcaacgcgtcagtgggctgatcattaactatccgctggatgaccaggatgccattgctgtggaagctgcctgcactaatgttccggcgttatttcttgatgtctctgaccagacacccatcaacagtattattttctcccatgaagacggtacgcgactgggcgtggagcatctggtcgcattgggtcaccagcaaatcgcgctgttagcgggcccattaagttctgtctcggcgcgtctgcgtctggctggctggcataaatatctcactcgcaatcaaattcagccgatagcggaacgggaaggcgactggagtgccatgtccggttttcaacaaaccatgcaaatgctgaatgagggcatcgttcccactgcgatgctggttgccaacgatcagatggcgctgggcgcaatgcgcgccattaccgagtccgggctgcgcgttggtgcggatatctcggtagtgggatacgacgataccgaagacagctcatgttatatcccgccgttaaccaccatcaaacaggattttcgcctgctggggcaaaccagcgtggaccgcttgctgcaactctctcagggccaggcggtgaagggcaatcagctgttgcccgtctcactggtgaaaagaaaaaccaccctggcgcccaatacgcaaaccgcctctccccgcgcgttggccgattcattaatgcagctggcacgacaggtttcccgactggaaagcgggcagtgagcgcaacgcaattaatgtaagttagctcactcattaggcaccgggatctcggctagctggccagggcccgatacgtcgcggtgagttcaggctttttcatatctcattgcccccggacgagcgtctgctccgccattcgccgtccgccgtgccaatcggatcagccgtccaaatgcgggattttcgttagtcggaggccaaacggcattgagcgtcagcatatcatcagcgagctgaagaaagacaatccccgatccgctccacgtgttgccccagcaatcagcgcgaccttgcccctccaacgtcatctcgttctccgctcatgagctcagccaatcgactggcgagcggcatcgcattcttcgcatcccgcctctggcggatgcaggaagatcaacggatctcggcccagttgacccagggctgtcgccacaatgtcgcgggagcggatcaaccgagcaaaggcatgaccgactggaccttccttctgaaggctcttctccttgagccacctgtccgccaaggcaaagcgctcacagcagtggtcattctcgagataatcgacgcgtaccaacttgccatcctgaagaatggtgcagtgtctcggcaccccatagggaacctttgccatcaactcggcaagatgcagcgtcgtgttggcatcgtgtcccacgccgaggagaagtacctgcccatcgagttcatggacacgggcgaccgggcttgcaggcgagtgaggtggcaggggcaatggatcagagatgatctgctctgcctgtggccccgctgccgcaaaggcaaatggatgggcgctgcgctttacatttggcaggcgccagaatgtgtcagagacaactccaaggtccggtgtaacgggcgacgtggcaggatcgaacggctcgtcgtccagacctgaccacgagggcatgacgagcgtccctcccggacccagcgcagcacgcagggcctcgatcagtccaagtggcccatcttcgaggggccggacgctacggaaggagctgtggaccagcagcacaccgccgggggtaaccccaaggttgagaagctgaccgatgagctcggcttttcgccattcgtattgcacgacattgcactccaccgctgatgacatcagtcgatcatagcacgatcaacggcactgttgcaaatagtcggtggtgataaacttatcatccccttttgctgatggagctgcacatgaaccaaaaggatctaggtgaagatcctttttgataatctcatgaccaaaatcccttaacgtgagttttcgttccactgagcgtcagaccccgtagaaaagatcaaaggatcttcttgagatcctttttttctgcgcgtaatctgctgcttgcaaacaaaaaaaccaccgctaccagcggtggtttgtttgccggatcaagagctaccaactctttttccgaaggtaactggcttcagcagagcgcagataccaaatactgttcttctagtgtagccgtagttaggccaccacttcaagaactctgtagcaccgcctacatacctcgctctgctaatcctgttaccagtggctgctgccagtggcgataagtcgtgtcttaccgggttggactcaagacgatagttaccggataaggcgcagcggtcgggctgaacggggggttcgtgcacacagcccagcttggagcgaacgacctacaccgaactgagatacctacagcgtgagctatgagaaagcgccacgcttcccgaagggagaaaggcggacaggtatccggtaagcggcagggtcggaacaggagagcgcacgagggagcttccagggggaaacgcctggtatctttatagtcctgtcgggtttcgccacctctgacttgagcgtcgatttttgtgatgctcgtcaggggggcggagcctatggaaaaacgccagcaacgcggcctttttacggttcctggccttttgctggccttttgctcacatgttctttcctgcgttatcccctgattctgtggataaccgtattaccgcctttgagtgagctgataccgctcgccgcagccgaacgaccgagcgcagcgagtcagtgagcgaggaagcggaagagcgcccaatacgcaaaccgcctctccccgcgcgttggccgattcattaatgcagctggcacgacaggtttcccgactggaaagcgggcagtgagcgcaacgcaattaatgtgagttagctcactcattaggcaccccaggctttacactttatgcttccggctcgtatgttgtgtggaattgtgagcggataacaatttcacacaggaaacagctatgacatgattacgaattcgatatcagggctacgctggaccggatgggctgagggagccgacggcacgcggcggctcacggcgtggcacgcggaacgtccgggcttgcacctcacgtcacgtgaggaggcagcgtggacggaattgtgagcggataacaattccggcgtcagagaagggagcggagcatatgacgcagtgcccgcgctgccagcggaacctcgcggccgacgagttctacgccgggtcctccaagatgtgcaaggggtgcatgacgtggcagaacctcagctacaacgcgaacaaggaaggccacgcgaacacgttcaccaaggccaccttcctggcctggtacgggctgtccgcgcagcggcactgcgggtactgcgggatctccgaagcggggttcacctccctccaccggacgaacccgcgggggtaccacatccagtgcctgggcgtggaccgctccgacagcttcgagggctactccccccagaacgcccgcctcgcctgcttcatctgcaaccggatcaagagcaacatcttctcggcgtccgagatggacgtgctcggggaggccatctcgaaggcgtggcacgggcgggggatcgcctagagatctccaatatgcggggatcgaccgcgcgggtcccggacggggaagagcggggagctttgccagagagcgacgacttccccttgcgttggtgattgccggtcagggcagccatccgccatcgtcgcgtagggtgtcacaccccaggaatcgcgtcactgaacacagcagccggtaggacgaccatgactgagttggacaccatcgcaaatccgtccgatcccgcggtgcagcggatcatcgatgtcaccaagccgtcgcgatccaacataaagacaacgttgatcgaggacgtcgagcccctcatgcacagcatcgcggccggggtggagttcatcgaggtctacggcagcgacagcagtccttttccatctgagttgctggatctgtgcgggcggcagaacataccggtccgcctcatcgactcctcgatcgtcaaccagttgttcaagggggagcggaaggccaagacattcggcatcgcccgcgtccctcgcccggccaggttcggcgatatcgcgagccggcgtggggacgtcgtcgttctcgacggggtgaagatcgtcgggaacatcggcgcgatagtacgcacgtcgctcgcgctcggagcgtcggggatcatcctggtcgacagtgacatcaccagcatcgcggaccggcgtctccaaagggccagccgaggttacgtcttctcccttcccgtcgttctctccggtcgcgaggaggccatcgccttcattcgggacagcggtatgcagctgatgacgctcaaggcggatggcgacatttccgtgaaggaactcggggacaatccggatcggctggccttgctgttcggcagcgaaaagggtgggccttccgacctgttcgaggaggcgtcttccgcctcggtttccatccccatgatgagccagaccgagtctctcaacgtttccgtttccctcggaatcgcgctgcacgagaggatcgacaggaatctcgcggccaaccgataatctagagactagtcaagcttcggatcctgcccgccgaacgcgtcgtcgtcgacggcctggtgctcatcgacgagcacccggagccaggtgaaaagcgccggcggacgctcggactgggcgcgggattccagcagtaacccaggtccgccggccacctcacggcaggcagaccctcggctttcgcgccgggaccgccatgagaccgccacccggatgtccggggtggcggtctcatggcggtccctcagcggccctacgcgaccgctgtgtcgacgcggaggcagtctccggggagccggccccagggctggagtaccggggcgagcttgcccttgcagcggcggcacacgggcgacgcggcgccgggcgggggagtcttgacgtcgacggtgaccggcttcggcttcaggcgcttccgaaggctgatcgtcgggcggatcgcctccttcttcggctgacgcactcggtcgagcgaagcggccagctcctccgtgcgggcctcgttggccttccggcgcgcctcgcggaaagcagcttcctcctcggacatgacctcgaacctcatctggtcagcgtcaaggtcgcccggcgcggccggcgcttccggggcgggcgggtccaggacgtccttgccccacaccaggccccaggactcgacgagccgccggacgcccggtaggccgtacgtctcggcgaccttgatgaggtcgaggcgacgtccggcgacgcgggcgatgtatcggtaccagatgtaggccgggatgaccgcgatggcgaccaggccctcggtgtcgtcggtgatctcctcctcggtgcggacgtcctgctggatgccgagttccttgatcagccggttcaggttctgcgaccggtagtgcttgcggacctggaagacgccgaactcgcgctcgcggtacttctcgacgaacgggccgggccgacgaagccgctgcagctcggcggccgccgcgtcgcccaggtcgagcggtcccatgcggtcgtcgccgcgaccggccttgaagttctgtccggccagctccaggccgatcttggcgacgccgcccttggtcttgtcgccgtccttgtagaggtagcgggcctgcttgcccgcatcgccgtcagcggcgtccgcgccgttgagtgggcgcacgtcggtgccgtggcccttgccctcacaggagcaaccgggccggtcgcacgtctcgctgacggtgtagccgcccgcggattcgaccccggcggcccaggctccggcgagtgcgtcgcggaacgcggcctgggcgtccgggccgagcacctcgcgggtgacccagagcgtgtgccagtgcaggtgccagccggagccccagccgaaggtgtcctcgaaggcccgctcgtagccgatgatcccgaagtcgtcgcgcatcgtgcgccagcggcggccggacgagccgtacgcgcccttccagccgtcgtgcaagaccgcgaccaggccgtgccgcattcccttgcggacggtgccgaacgccatgcgctcgaagtggcgcaacgtgttcgtgccaaggtgcagcccgtacccggcgtccgcgagaccgtcggcggcgagctgcacgttcgagccccgtacggccaggatgcggctcatgcaccacgggcaggtgtggacgttgttgcagcggcacgtgttgccccacgtcgcctcgcccggcttccacatcagctcggccgtcccggcagtgagccgggtcccgcagcccttgaacgcctcgttcagcgacaccgtctggtgccggtcccgccgggcgaaccgctcgtcgcgcgggtcctcccgcccggctgtcgcggcaccctcgtttggggtagaacccgttccagttacagcgctctgacctgcagtggacggagattttcccttactactaaagcccgcgtccggattacccgctgtagtcgtgcttgctacgctgcgtgactggtccgcaatgagacgctttgcgcgctttcggcaggcgtccgagcagtagattttggggcgcttcccggggatgtggacgatcggggtgccgcagtggcacttcggtccggcggggcgcggtggtgtcgacgcgctgttctctcgtacgctcgtcacagagcaaacgtcctcactcggcatgcctgcaggtc

SEQ ID NO: 39 - DNA, 30925 bp, synthetic construct
  source 1..30925: mol_type = other DNA
  misc_feature 1..30925: note = Actinorhodin biosynthetic gene cluster
ctgccgcacgacacaggagacgaaggcatgcgcgccgtacagttcgaccgttttggcccgcccgacgttctgcgcgtcaacgacgtccccgcgccccgacccgggccgggagaagtcctcgtcgaggtgcgcgccgcgagcgtggacgccggtgagaccgccttccgggcgggcaggatgcgccgggtgacccgcgtccgcttcccccgcggcctgggcagcgacttcgccggccgggtcgcggccctcggcagcggcgtacgcgcctggagcgtgggggacgcggtgtgggggctgatgccgcacctcaccttcggggcaatcgccgactacgtcgcggtgcccgagcagcggctggcccgggctccgcagaacctggacctgctcgaagccgccgccctgccggtggtgggcaccaccgcgatgacggccctgagcggcaaggcgcgactccagcccggggaacggctcctggtccgcggcgccaccggcggcgtcggcagcgtcgccgtgcagctgggcaaggcgctgggcgcgcacgtcaccgccctcgccgccgcccgcaacctcgactggatcacccggctgggggcggacgaggccgtggactaccgcacgacccggcccgaagacctcgaccggttcgacgtgatcgtcgacgtcgtcggcaccgacctgggtgcctaccggaagcggctggcccgcggcggacgtctggtcgccctctccttcgactcggaccgcgtcgtctcctccatgctcggcatcgccctgcgggcggccgccactccccggcgcgtcaagatgttcagcaacaacccctcggccgaccggatcgccgaactcacccgggccgtcgaggcgggcacgatccggccggtggtcgacaccgtcttccccatgcgggacatagcggcggtccaccagcggctcgaagccggcggcgtccgcggcaagtacgtcgtcgacctgcggcttccctagctcacggtcggccgatccccaggttcggcgcggcagcgcgtcagggtgtcagcgcgcactccgccgccgccacgaccgtgcgggcctggagttccacctgggcgtgcacggggacccagcgcagccgcagggacgtctcgaagtccgtgcaccaggcggtgaagagggcgtccagctcgtggtggagcccggcggcggccggggcgtcggccgcgtgcagcagccgcagcaggagtcccgccgcgcgtagcggctgacggcgcgcgacgacctccagggcgccgatccccgccgtcgtcaacgcgggtgagccgtcggtgcgcggtcccgcctccgcctgccggaccaggggcccccaggagtcggccaccaggtcgtacaggtcctcggccatccactccagtacgcgtacgggtgggctgtcctcgggtgccggcaggaggccgcgggccctctcgaacacggcggtcacctgccggccgccctcccgcaccagcccggacagcgcgcgcagggcccgggcggggtccgcgtgcggggtcgggtcgtccgccggggcggtggcccacagcggtacctcgacgatcgccgtggcaccgccgtaccgctggggcgcgcaccaggtggacaggccgatgtcctcggacccggccgccggccgcgcggtgctgcccggcggcggcaggacatggatgccgggggccggattctcccagtacagggcgtcgtacgtgccgtgctggaccgggacccccagggcggcggcggacgccgcgaagggggcggcgagtccggggaggtcgcgggtcagctgggcccaggtgccgcccgcgtcgacgttgtgcagggagcactggaggacggggcgcaggtcgtcgatcacgtcgaacagggcacggctctccgggagtggccggccgacgatcggggcccactccggctgctccgcggcgaccgggcggaaggcggcacggtagtacgacgccagggacggggcggggccggccgtcgcggtctcgatgccctcgctcagcgcggcgccgtccgggtcgaggcacaggacgatgtcccaggtgacggcctcggggtcggtcgccggggagcgccggtcgccgcctgcgaccagctccgccagcgccagtgccgtcgcgccgcccaccggctcgtccgggtgcggccgggccaccaccaggacgtgccggggtccgtggcccaccgacagcatcaggagcggccggcccgcccgggacgtgccgacacgacacaggcggccggtgcccgggaaacgggagaccagccgtcgcgccgactcggtgacctccgcgaccgtggggtatcggttcatcgggcgtgtccggtcaggctccgccgttgccgctctcgtccgccatgccgtctccttccgacggtgcccgtgggtacccgtgggtacctgtgctgcttttcgcgcctgtgctgcctgtggtgtgcgaggcgcgtcgtgccgctgtcagcgtccgttcaccggatcaccgctgtcaatggccggtgccgcccgcgcagtcgggggcggcgaagccggcgcgaaggcgagggtgcgcgtcaggccgggaagacgtggtcatgggtgacgtggcgggagcgcagcagcaactcgccgtccgccccccggaccaggacgtcgtgcacgaggcaactcggcccgaactccggcgccttgacgtcggcgtggacggtgagcaccaggcagtagctggtcgccgtgatcgagccgtcggacgcctggctcagcgccgtgtggtcgaaccagtgcctgcgctggattttgcgggcgtcgaacttgcggtggaagtcctccaggacggcggtgatcccggcacgggtgtgggcggcaggcagcgagggcgagtgcctgaactcgccgtcctcggtgaaggtcgcggcgtagccggcgaagtcacggccgtccagcttctgcatctggtggccgtagaacgacaggacctcggcgtacaggccggtgggaagcgcggtgatggtcatacggccacggtcgcccggtggcctcgaagttccctcgagccgggttcgagtgggcgctgccaggctcgtcgccatgagcaccgtgacagtgatcggggcgggcacgatcggcctgggatggatcaacctgttcagcgcccgcgggctgaccgtacgcgtcaacagccgtcggcccgacgtccggcgcgtcgtgcacgaggcgctcgagctgttctccccggggcgggtggacgagctggcggcgcgcatcgagtacgagccggacgtcggccgggcggtggccggggcggacgtcgtctccgagaacgcccccgacgacctgccgctcaagcagcggttgttcgcagagatcggagcggccgccccggaccacgccctcgtgctgtcctcgacgtcgaagctgcttcccgacgagctgagtcgggacatgccgggaccgggccggctggtcgtcgcgcatccgttcaacccaccgcacatcgttccgctggtcgaggtggtccgcggcgagcgcaccgacccggaggccgtcgaacggacactggccttcctggcgtcggtcgggcggacccccgtcgtggtgcgcagggcgctgcccggcttcgcggccaaccggctgcagtcggcgctgctgcgcgagagcatccacctcgtcctcgaaggcgtggtgaccgtcgaggagctcgaccggatcgtcaccgactcgatcggcctgcgctggtccaccatcgggccgttccacgcgttccacctgggcggcggtcccggcggcctgcgcaagtggctcgagcacctcggcagcggcctcgaacagggctggcgtgggctcggacagcccgccctcaccccgcaggccgtcgaggctctggtcgcacagaccgaagccgcctacggacaccggccctacgccgaactggtccgggaccgtgacgaccggcacctcgccgtactggccgccctggagcggaccgagcagccccaggaggagaccaagtgatgcgtgccgtgcagttcgaccggtacggggaccccgacgtgctgtacgtcgccgagcgtcccgtccccgaacccggccccggccaggtgagaatcgccgtcgacgccgtgagcgtcggccacgcgcagacccagatgcggcgcgaggccttccccgcgccgatgtggcggcccgtcttccccgtcgtcctcggcggcgacgtggtcggcaggatcaccgcggtgggaccgggcgtcacggccctgcggccgggagaccgggtcggtgcgttcaccctctacggcgcctacgccgagcaggtcgtcgtcgacgccgtcaccgtcgtacccgtgcccgaggagctggacgccgccgaggccgcggtcctcccgggcaccggactgatcgccctcggcatcctgcggaccggacgactgcgcaagggcgagacggtgctgatccacgcggcggccggcggggtgggccacatcgcggtccagctcgcccgggcggccggcgccggcctgatcatcggcaccgcgggcgcggccgccaaacgcgagttcgcccgcgcgacgggcgccgacgccgtcgtcgaccaccgctccgcacactgggccgacgaggtccgggaactcaccggggggcgtggccccgacctgatcctggacggcatcggcgccgaggtcctggagcagggagtcggtctgctcgctccgggcggccggctggtgttctacggctcgtccggcggcgagctggcgatcccgaaggtgtcggtgatggacctcatcggcatcaagtacgtcaccggcttcgccctgtcggcctggcgcggtggccgcccgcaggagtacgaggcgggcgtcgccgaactcacccgactgctggccgaaggacaggtcacgtccgcggtgcacgcccggctgccgctggagcgggcggccgaggcgcacgccgtcgtcgaggccagggcccagctgggccgggtcgtgctcgtcccctgaaacgaccaggcattcctccgaagtgtccaagcattcctgatccaagagcccgaaggagacctttccatgacctcgtcgctgcaccacgcgatacgtctgaccaccgcgtccgccatcgccctgggcggactcgtgaccctggggaccagcgcgcacgccgcgagcgtcgccgtgccgtacgagtgccgcacctgggtgcagggcaacacgcacccggtctacgactacgcgcgcggcttcgacgtcagcgtgcccgcctcggtccgcgcgggcaagaagttcaaggccacctacgatcccgacccgatcaccgccttcgccgagtacaaccagatcgtcaacgacgtgcggatcgcctaccggatcccggacggcgcgaaggtccacaaggtgcggctcaccggcggcagcggtctcggcgactccgacgtccgggtccaggtcaagggccgggacatcgtcgtcagcgcctccggccccttccagggcggtgtcgagttcgacctgccgacgctgaaggtcacctacaaggcgccgaagaccaccggcccgctcaacttcgtctcgggcggctcgggttacgaggaccccggcttctactggtaccgctaccagccgatcctggacgagtggggccccttcgagtgcttccccgacccggcgaagcccgaggccgtcctggccagcacccaggtcaagaagcacaagtagacacagcggggtcggacgaacaatggagaacgcatgcccaaggccgtagccatccaccagttcggcgggccggacgtactgggcctcgtcgatgtccccgagccggtgccgggaccgggccaggtgaccgtccgagtgcgggccgccggagtcaacgggttcgactgccgggtgcgctccggcggcatgcgcggtcgctatccggtcgagttcccgcagatcatcggcaacgagttcgccggggtcgtcgagcggaccggaccggaggcgaccgggttcgcgcccggcgacgaggtgctcgggttcgccgtgcttcagtccggcaccgagctgctcgccgtcggcgcggaccagatcaccgtgaaaccgccggagctgtcgtgggaggtcgcgggatccctctcggccgtcggacagaccgccgacatcgccctggccgaactgcgggtcggccccggggacaccgtgctcgtgcacgccgcggccggcggcgtcggcagcctcgccgtccagctcgtccgggagcggggcggcacggcgatcggcagcgccggcgagcacaaccacgactacctgcggtcgttgggcgcactgcccgtcgcctacggcccgggcttcgccgaccgggtgcgggccctggccccgaacggcgtcgacgccgccctcgactgccacggcggaccggaagccctcgccgtgtcgctcgaactcgtcgcggaccgggcccggatcgccaccgtcgccaacttccgcgccgcggcccaggagggcatcgtcatgccacgggtggtgcggtccgccgagcggctcgccgcgctggccgcactctgcgccgagggccggctgcggccgcacgtcgaggccgtcctgcccttcgccaaggcggccgaggcccatcaccggctggagcagggccatgtccggggcaagctcgtcctggtgccggacctgtgacggcgaaccccggccgtccgggcggcccggcggaccagggccacccgcgccgctgggccatcctcggggtgctggtcctcagcctggtcggcatcatcctcgacaacaccgtgctcaacgtgacgctgcgcaccctcaccgaccccgagcagggcctgggcgcctcgcacagccaggtggaatgggtgctcagcgcctacaccctggccttcgcggcgacgctgttcacctggggagtgctgggcgaccgactgggccgcaggcgggtactcctgctgggcctcggcctgttcggactgtcgtccctggccggggcctacgccgggtcgccggagcagctcatcgccgcccgtgcctgcatgggggtgagcggcgcggcggtgctgccgagcacactcgccaccatcgccgccgtcttcccgctgcgcgagcggcccaaggccctcgggatctgggcggcctcggtcggcttcgccctcggcatcgggcccgtcaccggcgggatactgctcgcgcacttctggtggggctcggtcctgctggtcaacgtgcccctcatggccgggtgcctggtcgcggtggtgctggtggtgcccgagacccggggcacggcgggcaggcgcgtcgacgcggccggactgctgctctcgatcgcgggtgtcgtgccgctcgtctacgcgatcatcgaggccggccggagcggcggggtcacccggcccgcggtctgggcagccggcctggcgggcctcggcctgctcctcgtgttcctgtggcacgagcgccgtaccccggaaccctcgctggagctcggcttcttccggatgaaggccttctccaccgccgtcgcggccgtcggcttcgtcagcttcgcgatgatgggcttcctcttcttcagcgccttctacctgcagagcgtgcgcggctacacacccctgcaggccgggggatgcaccgtggcactggccgtcgcgaacgtggtctgcggaccgctcagcacggtcctggtgcgttcgatcggcccccggaacgtgtgcgcggcgggcatgctggccgtcaccgcatcgctctgcggggtcaccttcgtgacccagcacgcacccgtatggctgatcctcgtcctgttcgccgcgctgggggcgggcgtagcatgcgtcatgccgaccgcggccgtgtccatcatgaacgcgatcccacgcgagaaggcgggcgtcgcctcggcgatgaacaacaccgtgcgccagctgggcggcgccctgggcgtcgcggtgctcggttccctcatgggcgccgcgtaccgccgcggcatcgaggacgagctcgccgtactgccgccctccgcgcggcaccaggccggcgagtccctggatgccaccctgctggccgcgactaggctgggggagagcggacttgtcggccccgcgcgccaggcattcctggacgccatgcacctggccgccggggccgctgccgcggtggcgctcgtgggggcccttgccgtgctccgctggctgccctcctccgtcacgactccgacgcccccggcaggggccgtgcccggccgggagcattccgatcacctcaaggtccaaggaagctgacatgcctttcactcctgacgagctcgagtactacgcctcccagaacctcggccggctggccaccgtggcgcccgacggccagccccaggccaacccggtctcgttccgcgtcaacaccgagaccggcacgatcgacatcggcgggcacaacctgaccgccagcaagaagttccgcaacgtcaccaagcacgaccaggtcgccttcgtcgtcgacgacctgatctccacgcagccgtggaacgtacgcggtatcgaagtgcgcggccgggccgaggcgctgaccgacgcgcagccgccgcacccctacttcggtaccgcgatgatccgtatccaccccaagcgcatcatcacctggggcctcggcggcgacgccgcccagcgcggccgcgacgtctgacccagcacccttcgactccgcttcgagcggacctcgacgccctcttgccaaggtggagcccgtaggacgggtacaccacggggagggcggctggatgagtacagagatcttccatgaggagttcgccggggggctggtgaccgaggggccgggcgcgccgtggcggcttcgcccggtcgacggtctcgaggcgggagacgggctggtccgcgggggaccggacggcctggtggtcgtgccgagcgccgcccacccggggacccggcggccggcgttcaccgagcccaagcccgggccggacggcaccccgctgcatctgcggtggggtgccttcaccaccggcggcaccaccggcggcaccgccggcgcgcgggcggcgttcaccgccgtgcccggcgaacggctctcggtcagggccgagatggggctgcgcggcttcggtctgcgctcccatccgtacgacgacgtgaccgaacccgacgcggacgcccggctcggcgcgggcggtctgatctcggtcgatctcgagtccgggatcatcttcgacttcttcctcacacacagccggctctacgcggtctacgagcggctcgcgctgcggccggacgccgagttcgcggccttcacctactgcgtcccggtcgcggaccgcacccccggcacgctccaccggctcgaggtcggatacgacgtcgcggccggcaccgcccactggacggccgacgggcaggaggtcctgtccgtggaccggatcggcttccgcgcactggacgcgcgctggctccggcgggacaacggcggccgcgaggaggccgtacggccgcgcggactcagcttcggcctcgggctcttcctggagcgccacttcggccagggggtgcggctgtcggtgcgaaggctgtcggtgctcacctcgcccgccggctcccgcgactcgtgacgacgaccaacgaaaggcactgcgatgcccgatgagaacaagcccgtactggtcctcggcgccaccggaaagcaaggcggctccgcggcccggtacctgctggaacgcggctggacagtccgggccttcgtccgggaccccggcgcgcccaaggccaaggagctgcgtgagctgggggcgagcctgcacaccggcgacctggaggacgccggctcggtgcgcgccgcgatgaagggtgcgtacggcgtgttcagcatccaaacgccgatgacaccggccggcgtggagggcgaggagcggcagggcaagatatgcgccgacgccgcccgcgacctcggcgtccagcactacgtccacagctcggtgggcggcgcggaacggccggagggcgtgaactggcggctgtccaagctcgcgatcgagcagcggatccaggagaacgcgctccggttcaccttcctgcggccgtcgtacttcatggagaacctgaaccacgacatgtcgcccctcgtcatggaggacggcgtgctgaccttccggagggggctcgggccggccaacaccctgcagatgatcagcggccccgacatcgggtacttcgcggccgacgccttcgacgaccccgacaccttcggcggcgccaagatcgagctggccggggacgagctgaccggcgagcagatcgcggccgcgttcggccggcacaccgggctgcccgcccgcttcgtgtcggtgccgataccggagctgcaccgcacggggttcgagtggcaggcgatctcgtacacctggctcaacggcatcggctatcacgccgacatccccacgctgcgcgcccggttcccgcagctgctcaccctcgaccagtggctggccaggaccggctggaccccgagggacccggcatgagcgaggacacgatgacccaggagcggccgtccctgacggcacacgcccgccggatcgccgaactcgccgggaagcgggcggccgacgccgaacagcagcgccggctgagccccgacgtcgtcgacgcggtccttcgagccggtttcgccgcccacttcgtaccggtggcgcacggcggccgggccgcgacgttcggggagctggtggagcccgtcgcggtgctcggcgaggcctgtgcctcgaccgcctggtacgcctcgctcacggcgagcctcggccggatggccgcctacctgccggacgagggccaggccgagctgtggtccgacggccccgacgccctgatcgtcggtgccctgatgccgctgggccgggccgagaagaccccgggcggctggcacgtgtcgggcacctggccgttcgtcagcgtcgtggatcactccgactgggcgctgatctgcgccaaggtcggcgaggagccgtggttcttcgcggtgccgcgacaggagtacgggatcgtcgacagctggtacccgatgggtatgcgcggaacgggcagcaacacgctcgtcctcgacggggtgttcgtgccggatgcgcgggcctgcacccgtgcggccatcgcggcaggtctcggtccggatgccgaggcgatctgtcacaccgtgcccatgagggcggtcaacgggctggccttcgcactgccgatgctcggcgcggcccgcggggccgcggccgtgtggacctcgtggaccgccggaagactggccgggccgaccgggcagaacgccgtctcgtcccaggaccgcgtggtgtacgagcacacgctggcccgggccacgggtgagatcgacgcggcccagctgctgttggagcgggtcgcggcggtcgccgacgccggctcggcgaccggcgtactggtcggccgcggggcgcgggactgcgccctggcggcggagctgctgaccgccgcgaccgaccggctgttcgcctcggcgggcacccgggcacaggcccaggacagcccgatgcagcgcctgtggcgcgatgtgcacgcggcgggcagccatatcgggctgcagttcgggcccggggcggcgctgtacgccggagagctgttgaggaggagcaacgatggctgaagtgaacgatccccgggtgggcttcgtcgcggtcgtcaccttcccggtggacggccccgccacccagcacaagctggtggagctggccaccggcggggtgcaggagtggatccgcgaggtgcccggcttcctgtcggccacgtatcacgcgagcacggacgggaccgcggtcgtcaactacgcccagtgggagagcgagcaggcctaccgggtgaacttcggcgccgacccgcgctcggcggagctgcgggaggcgctgagctcgctgcccgggctcatggggccgccgaaggccgtgttcatgactccgcggggggcgatcctgccgtcctgacctggtcgtccgcggcctcgccggccccggccagcaggccggcgatgatgatctcgaggccgagctcgaaccggcggtcggagtcgagcgaggtgatcgggccggccaggtggaccaggttcgggaaactggtggccggcagtgacttcaggtagccgtggagctggtcggcgaacacgccggcctgctcccggccctgttccgttccggggttgcgggacgactgctccagggcctccgccgtgacgaaggtcgacagcaggtcgcccccgtaggcggcgagttcgtcgtgcaggcccccggagcgcagcaggttcatggtgcgctccatccccaccatcccgttgggtcccagcggcacccggtcgatcgcgatccgtgccaggtcccggtgggccaggaacatcctccgcagcgaccggcacatctccttgacctgctccgcccagcggccgggttccggttccgggacctccacctcggtcagcacgatgtcgaagacgaggtcgagcagctcgtcccggttccccacgtgcgcgtacagcgaggcgtgtccggtcttcagctcctgcgcgagccgccgcatgctcagggcgtcgagtccctcggcgtcgaggatgccgagcgccgtgacgacgatccggtcctgggtcaggggcatgcgcggcggcgccttcttcggccggcgccacggaggcacgggaatctcctcgggcatgggcctcccttcctcgcttcgcgacacgtgctcctcatcgtatggcatgaacgggccaccgtttcttgacgcgaccaccgttccattgtagaacggtggtcgttcgtggaccaatagtcgaggacccgggggacgccatgagttccgttgaagccgacgagccggacagggccacggccccgccgtcggcgttactgcccgaggacggccccggaccggacggaaccgcggccggacccccgccctacgcgcgccgttgggccgcgctgggagtcatcctcggcgccgagatcatggacctgctcgacggcacggtcatgaacgtggccgcgcccgccgtccgcgcggacctgggcggcagcctcagcgtcatccagtggatcaccgtcgggtacacgctcgcgttcgccgtcctgctcgtggtgggcggccggctgggcgacatctacggccgcaagcgcatgttcgtcgtcggcgccgtcggcttcaccgcggcctccgtgctgtgctcggtggcggccggtcccgagatgctcaccgcggcacgcttccttcagggcgggctcggcgcgctgatgattccgcaagggctcggtctcatcaagcaaatgttcccgcccaaggagacggcggcggcgttcggcgcgttcggacccgccatcgggctgggcgccgtgctcggcccgatcgtcgccgggttcctggtcgacgccgacctgttcggcacgggctggcggtccgtcttcctgatcaatctgccgatcggcgtggccgtgatcgtcggcgcggtcctgctgctgcccgagggcaaggcgcccgtgcggccgaagttcgacgtcgtcggcatggcgctggtgacgtccgggctcaccctgctcatcttcccgctcgtccaggggcgcgaacgcggctggcccgcctgggcgttcgtgctgatgctggccggagcggccgtgctcgtcggcttcgtcgcccacgaactgcggcaggagaggcgcggcggcgccacgctcatcgagctcagcctgctgcgcaggtcccgctacgccgcgggactggcggtggcactggtgttcttcaccggcgtctccggaatgtcgctgctgctcgccctgcacctgcagatcggcctgggcttcagccccaccagggccgcgctgaccatgacgccctggtcggtgttcctcgtcgtcggcgcgatcctgaccggggcggtgctgggatcgaagttcggccgcaaggccctgcacggcgggctcgtggtgctggcgctgggcgtgctgatcatgctgttgacgatcggcgaccaggccggcgggctgaccagctgggagctcgtccccggtatcgccgttgccgggctcggcatgggcatcatgatcggactgctcttcgacatcgccctggccgacgtcgacaagcaggaggccggtaccgcctccggcgtcctcaccgcggtccagcagctcggcttcaccgtgggcgtcgcggtgctcgggaccctgttcttcgggctgctcggctcacaggccacggcgagcgtcgacgacggcgcgagccgggcccgcaccgaactcgccgccgccggggcgagcacgaccgagcaggaccggctcctggccgacctgcgggtgtgcctgcgggaatcggcgagtcagcaggactccgaacggacgccggacagctgccgaaacctccagcaggcccggccggcggtggccgaggccacggcgcgggcctggcggacggcccacaccgagaacttcagcaccgcgatggtccgcacgctctgggtggtgatcgcactgctggcggtctccttcgcgctggccttccggctgccgcccaagccgcgtgaggaagagggcttctgatgacacgcacactgctgtcctggcccggcggacgccggctcaagtggctggtgctcgcggcctggatcggtctgctgatcgtgctccagccgctggcagggaagctcggcgacgtcgagtccaacgacgccgccgcctggctccccggcaatgcggagtcgaccgaagtgctcgagctgtccgagaagttccagccggccgacaccagcccgaccgtgatcgtctacgaccgcccgtccgggatcacggccgccgacgaggcgaaggcgcgggccgacgccacgcacttcgcggacggcaccggtgtggtgggcgagccctacggcccggtgcgctcggacgacggcaaggccctgcgcaccgtcgtcaacgtccacctcggcaaggacggctgggaggggctcaacgcggccgcgaaggacatgcgggcgatcgcccggccgagcgccccggacggtctcggcgtccacgtcacgggtccgaccggttacgccgccgattccgcagagtccttcagcagcgccgacttcaagctcaccctggtcaccctcctcatcgtcgtgacgatcctcgtcgtcacctatcgcagtcccttgctctggctgctgccgatgatctccgcgggcatgtccctggtcatctcgcaggccatcgtctacctgctggccaagaacgcgggactcacggtcaacgcccagacggcgatgatcctcacggtcctggtgctcggcgcggccaccgactacgcgctgttgctcgtcgcccgctaccgcgaggagctgcggcggcacgaggaccggcacgaggccatggccgtggcgctgcgccgggccggtcccgccatcgtggccagcgccgccaccgtcgccgtcagcatgctcgtcctgctgctggccgctctgaactccaccaagggtctcggcccggtctgcgccgtcggcgtgctggtcggcctgctgtcgatgatgacgttgctgcccgccctgctggtgatcttcggacgctgggtcttctggccggcccggccgaagcacggtacggagcccgacgtcacccggggtctgtggtcgcggatcgcccggctggtgtccggccgtccgcgtgccgtctgggtcaccaccagcctgctgctgggggcggtggccacgctggccgtcaccctgaacgccgacggcctccagcagaaggacggtttcaagaccaagccggagtcggtggtgggcgaggagatcctgacccggcacttcccggccggctccggtgaacccatggtcgtcatcgccaagggcgcctcggcggaccaggtgcacgcagctctggagaccgtgcccggcgtcatcgaggtcgcaccaccacaggtgaaggacggcctcgcctatgtcgaggcgacgctcggcgccggggcggactcgccggcggccatgcgttcggtcaccgcggcccgcgagacactcgcccggctggacggtgcgcaggcacgggtgggcggcagcagcgccgtcgtgcacgacatgcgggaggcgtccagccgcgaccgcggtctgatcattccggtgatcctcgccgtggtgttctgcatcctcgcgctgctgctgcgagcactggtggcgccgctgctgctgatcgcgagcgtggtgctgtccttcttcaccgcgctcggcctcgccgccctcttcttcaaccacgtcttcgacttcgcgggagccgattcggccttccccctgtgggtcttcgtcttcctggtcgccctgggcgtcgactacaacatcttcctcgtcacccggatcaaggaggagagcgaccggctcggcacccggcagggcgcgctcaagggcctcacctcgaccggtggcgtgatcaccgcggccgggctggtgctggccgggaccttcgccgcgctggccacgctgccgctggtcttcatcgccgagctcggattcacggtcgcggtgggcgtcctgctcgacaccatgatcgtgcgatcggtcctggtcaccgcgctcactctcgatgtcggccggtggatgtggtggccgcacccgctcgcccggcgcgaggacccttccgaggacccagccgtatcaggaatgccagattctattgattcggaagcctcgaccactgcctctcggtaaaatccagcaaaaattaatcagtgcagctcgctgcactgattaatttttgatcaataggagatcgcttgtgacggcaagcacattgaaatctgttgagtaggcctgttattgtcgcccccaggagacggagaatctcgacgggggcgcagatgagattcaacttattgggacgtgtccatgtaatcaccgatgcgggatgtgtaattccgcttaaatcctcgaaggcgacccagctcctggtgctgctgctcctcaggcggcacgaggtggtgggatcgggggtgctcatcgaggagttgtgggcggaccacccgccccgcagcgccatgacgacgctgcagacgtacgtgtaccacacccgccggctgctgggggagcaccgggtgacgagcgacgaccgggaattggtcctgacccagccgcccggctacttcgccctgatcgacgaggacgaactcgacgtcgcggtcgccgagcgtctgatccgcaccggcggccggctgctcgaggagaaccggctcgaggaggcgctcgcctcgttggacgcgggactggatctctggcgaggcccggcgctgtccaccgtaccgtgcggccgggtgctcgaaagcaatatcgcgcacctggaagagctgcggctttttggaatgcagctccgtatcgacgcgaattggcggctgggcagaatagggccgatgattccggaactccggtccctggtaatttcgcatccgctgaacgagaccctgcacgccaaactgatgggcgcgctctgtcagatgggcaggcgcgccgaggcgctggaatcgtatcggaatctccggcggatactgtccgacgaactgggggtggatccgacgccggaaatccagcgtatgcacatggaaattctcaacggtgagaaggtgctcgtgtagcaccggtccgtgaacgcggtggagcccctcgcagcctgcgaggggctccaccgcgttcacggaccggccggcgtcagtagttccccagcccgccgcagacgttcagcgcctgcgcggtgaccgcggccgcaccgggcccgatcaggtacgccaccatctccgccacctcggacggctgcacgtaccggccgatcggcacgcgcgcggtgatccggtcgaaggcctcctcggtcgacacctcccagatgtccgagtagtgctcgcgcacggacgcggccatcggcgtctcgacgaatccggggcagacggcgttcaccgtgatgccggtcctcgccagttcgagaccgagcgccttggtgaagccgaccacgccgtgcttcgaggcggagtagggcgcggcgtgcaccacaccctgctttccgccggtcgaggcgatgttgacgattcggcccgtgccccgttcgagcatgccgcccgccttgaggacctgtttggtcacccggaacacgccggtgaggttggtctccacgacatcgagccagagttcgtcggcgagttcggccgtggcgccgccgccgggccggcccgcgttgttcaccagcacgtcgaccggaccgtaacgctcgaccaccgccgccacgagagcctcgatctccgggaccgagcggacgtcgcaggtccgcccgtccgcctccacgcccgcctcccgcaactccttcagcgtcgtccgcagtccttcttcgccgcgcgcgcagacgaacacgcgcaacccctccttaccgagcctgcgggcgatctccagcccgattccgctggtcgcacccgtcaccagtgcgacttcggagtcctgcgtggccatgtgttcccctccctgcctcgtggtccctcacgcgctcagctttgggcgcccggctcgagcggcggtcgaagggagatggggtgccgctggacgcggcgccggtggatccggcatcgaggggtcccgtatcggccttcgagcctccttcgagccacggggccgacgatgacgacgaccaccggacgaacgcatcgaaggagctgttcggattgaagcgcagagtcgtcatcacgggcgtcggcgtccgcgcccccggcgggaacggcacccggcagttctgggaactgctcacctcggggcggacggcgacgcgccggatctcgttcttcgacccctcgccctaccgttcacaggtcgcggcggaggccgacttcgacccggtcgccgagggcttcggcccgcgggagctcgaccggatggaccgggcctcgcagttcgccgtggcctgtgcccgggaggcgttcgccgccagcgggctcgacccggacaccctcgaccccgcccgggtcggggtcagcctcggcagcgcggtggcagcggcgaccagcctggagcgcgagtatctgctgctgtcggactccggccgtgactgggaggtcgacgcggcctggctgtcccggcacatgttcgactacctggtgcccagcgtcatgccggccgaggtcgcctgggcggtcggcgccgagggcccggtcacgatggtctccaccggctgcacctcgggcctggactccgtcggcaacgcggtccgggcgatcgaggagggcagcgccgacgtgatgttcgcgggagccgccgacaccccgatcaccccgatcgtcgtcgcctgcttcgacgcgatccgcgccacgacggcgcgcaacgacgacccggagcacgcctcgcggccgttcgacggtacgcgggacggcttcgtgctggccgaaggagccgcgatgttcgtcctggaggactacgacagcgcgctggcccgcggagcccgcatccacgccgagatctcggggtacgcgacgcgctgcaacgcgtaccacatgacgggcctgaaggccgacggccgcgagatggccgagaccatccgggtcgccctcgacgagtcccgcacggacgcgacggacatcgactacatcaacgcgcacggctccggcacccggcagaacgaccgccacgagacagcggcgtacaagcgcgccctcggcgaacacgcccggcgcactccggtcagctcgatcaagtcgatggtcggccactcgctgggcgcgatcggctcgctggagatcgcggcctgcgtactcgccctcgaacacggcgtggtgcccccgaccgccaacctgcgcaccagcgaccccgagtgcgatctcgactacgttccgctggaggccagggagcggaagctgcggtccgtactcaccgtgggcagcggcttcggcggcttccagagcgcgatggtgctgcgcgacgccgagaccgcgggggcggccgcatgagcgtcctcatcaccggagtcggcgtcgtcgcacccaacggcctcggcctggcgccgtactggtcggcggtgctggacggccgccacggcctcggcccggtcacccgcttcgacgtgagccggtacccggcgaccctcgccggccagatcgacgacttccacgcgccggaccacatcccgggccggttgctgccgcagacggacccctccacacggctcgcgctgaccgccgcggactgggccctccaggacgcgaaggcggacccggagtcgctgaccgactacgacatgggcgtggtgaccgccaacgcctgcggtgggttcgacttcacccaccgggagttccgcaagctgtggtccgagggccccaagtcggtcagcgtgtacgagtccttcgcctggttctacgcggtgaacaccggccagatctccatccggcacggtatgcgcggtccgagcagtgccctggtcgccgagcaggccgggggcctggacgccctgggccacgcccgccgtacgatccgccgcggcacgccgctggtggtctccggcggggtggactcggcactcgacccgtggggctgggtctcgcagatcgccagtggccggatcagcacggccaccgatccggaccgggcgtatctgcccttcgacgagcgggcggccggctacgttccgggcgagggcggggccatcctcgtcctggaggacagcgccgcggccgaggcccgcggccggcacgacgcgtacggcgaactcgccggctgcgcctccaccttcgaccccgcccccggatccggacggcccgcgggcctggaacgcgcgatccggctggcgctgaacgacgccgggaccggtcccgaggacgtcgacgtcgtgttcgccgacggcgcgggcgtgcccgagctggacgccgccgaggcccgggcgatcggccgggtgttcggccgcgaaggggtgcccgtcaccgtccccaagacgacgacgggccgcctctactccggcggcggcccgctcgacgtggtcaccgccctgatgtccctgcgcgaaggggtgatcgcgccgaccgcgggcgtgacgtccgtaccccgggagtacggcatcgacctggtgctcggcgaaccccgcagcacggccccgcgcaccgcactggtcctggccaggggccgctggggcttcaactcggcggcggtcctgcgccgtttcgcaccgaccccgtaacgaccccgagaactggagaaagccatggcaaccctgctgaccaccgacgatctgcgccgcgccctcgtggagtgcgccggtgagacggacgggacggacctgtccggcgacttcctcgacctccgcttcgaggacatcgggtacgactcgctcgccctgatggagaccgcggcgcgactcgagagccggtacggcgtgtccatacccgacgacgtcgccggccgcgtcgacacgccgcgagagctgctcgacctgatcaacggcgcactggccgaggcggcatgagccggccgggagaacaccgggtggtccacaccctgaggacccaggccccggcgcggcggctctacgagctggtcgcacgcgtcgaagactggccggccgtcttcgaacccaccgtgcacgtacaggtcctggagcgcggcccgggcaccgaacgcttccggatctgggcgcgcgtgggcggccgggtgaagacctggacgtcccgccggacgctggatcccgacaccctgagggtgacgttccgccaggagctcacccagccgcccatcgcctcgatgggcgggagctgggagttccggggcgacggcgacggcaccgaagtcgtgctgacccacgacttcgccgcggtcgacgaagccgccctgccgggactgcgcgaggcgctggacgcgaacagcgggaaggagctggccgcgctggtcgcgctggcggagcgccggcagccgcccgaggagctggtcttcacgttcgaggacacgctccgggtgccgtccggggacgacgcctacgccttcatcgagcgcagcgacctgtggcaggaacggctgccgcacgtgcggaaggtgacactcaccgaggaggcggcgggtaccggccccgccgagacgcgggacatgaccgtccaggacatgaccatggagacggtgaccaccgacggcggtacccacaccacccgttcgatccggctctgcgtccccgcgaggagcatcgtgtacaagcagctcgtcccgcccgccctgctctccgggcactgcggcgcctggaccttcggcgaggacacggtcaccgcccgccacaccgtggcgatcgacccggcccgcgtggaagaggtcctgggcaaaggcgcgaccgtcgcggacgcccgtacccatctgcgcgaggtgctcggtgccaacagccgggccacgctccgccacgcggcggccgccgccgggccggcgtcatgacggtcgaggtccgtgaggtcgccgagggtgtctacgcctacgagcaggcccccggcggctggtgcgtcagcaacgcgggcatcgtggtgggcggcgacggcgcgctcgtcgtcgacacgctgtcgacgatcccgagggcgcggcggctggcggagtgggtcgacaagctcgccgcgggccccggccgtaccgtggtcaacacccacttccacggcgaccacgccttcggcaaccaggtcttcgcgccggggacgcggatcatcgcgcacgaggacatgcggtccgccatggtgacgaccggcctggccctcaccgggctctggccgcgggtcgactggggcgagatcgagctgaggccgccgaacgtgaccttccgcgaccggttgaccctgcacgtcggcgagcgacaggtcgaactgatctgcgtcggccccgcgcacaccgatcacgacgtggtggtctggctgcccgaggagcgggtgctgttcgcgggggacgtcgtcatgtcgggcgtcactccgttcgccctcttcggttcggtggccggcacgctggccgcgctcgaccggctggcggagctggagcccgaggtggtcgtcggcgggcacggcccggtggcgggacccgaggtgatcgacgccaaccgggactatctgcgctgggtccagcgcctcgccgccgatgcggtcgaccgccggctgacaccgttgcaggccgcgcgccgggcggacctcggcgccttcgccgggctgctggacgcggagcgcctcgtcgcgaacctgcaccgggcccacgaggagctgctgggcgggcacgtgcgtgacgccatggcgatcttcgcggagctggtcgcctacaacggtgggcagctgcccacctgcctcgcctagggagttcgaagatggcagccgaccagggaatgctccgggacgccatggcccgggtgccggccggggtggcgctcgtcaccgcccatgaccgcgggggagtcccgcacggtttcaccgccagttcgttcgtgtccgtctcgatggagccgccactggcactggtctgcctggctcgtacggccaactccttcccggtgttcgacagttgcggcgagttcgcggtgagcgtgctgcgcgaggaccacacggacctggccatgcgcttcgcgcgcaagtccgcggacaagttcgcgggcggggagttcgtccgtaccgcgcggggagcgaccgtgctcgacggagcggtcgcggtcgtcgagtgcacggtccacgagcgctacccggcgggcgaccacatcatcctgctcggcgaggtccagtccgtgcacgtcgaggagaagggcgtaccggcggtctacgtggaccgccggttcgccgccctgtgctcggcggcgggtgcctgcccgtccgccaccgggcggggcgtgcccgcgcatgccggctgaggccggccgggaaggccgtcagcggcccgtggcaccgtcgatcagctcgcggaggatgtcggcgtggccggcgtggcggccggtctcctccaccatgtgggtgagggcccagcggacactgggcgcggggcggcccggtcgcggccgggggagcggtgcgccgaggtcggtgcaggcgtcgagcacgcggttcgcccgttcgacggcctcccggtagcgggcgacgacgtcggcgacgccgtcctgggacgcggcccggaacgtcgccggccagcttcgcacctcctccccgaggaagaccgcgcgctcgacgtgggtcaggtggttgagcagcccgagcaggttggtgccggacgccaccgccgccgtgcggacctgcggttcgggggcgtcctcgaccttgccggcgatcgaggtccgcaggtagtcgaggaacccgcgcagggtctcggcctcaccgccgccggttcggggcggcggggtgtcccggcggtgggtgcggggggtggtgggcatggtgaccggcctccggaaggtgtggggcgggcgggccgcgggcgcggggcccgtcagtccgcgcggcggacgagcaggacgtggtcgacgacctcggcggtgcgcccgcccgggccggtcgcggtccggcgtggcgcctcggcccgttcgacccgccacgtcgccgggtccagggcgaggtccgccgcgacctcctgcggggccgggtggcgcgcgtcggggtcctggtcccacgaccacggcgccgtcgagccgtggtcgacgaccagcagccgcccgcccgggcgcagcgcgtgcgcggccccgcgcaggaccgacgcgcggtccaggtcgaagggcgtgtggaggtagtgcgcgctgaccaggtcgaaccggccctcggggaaggagtcgcgcaggtcgtgccgcacggcgtcgaccaggtcgccgaggccgtgggtccgtgcgtgccccgcgagccgctcggccgcgaccccggagatgtccacggccgtgacccgccagccccgccgggcaagccacagcgcgtcgccgccgctgccgcaccccaggtccagggcgtcgccgggcggcaggccggtgaccgtctcgaccaggcggacgttcgggcggggcgcgtcgggcgccgggcgggcggcgtacacgccgtcccagaacgtgaccgcgtcggtggtgctcatcggaactccttcagtcgtttcggccggcggcgggcgacgagtcgggcaacgcgccgcgagccgtcgatgcgaccagtctcgacaccctccgcccgaaccggcacgaaaacttgcggttgtggcaaggtggcccgatggacgccgcaacggacgacgtgctcgacgccgtgggcccacgcctgcgcacgctgcgccgcgagcgcggcatcaccctcgcccacctctcggcggcgaccggggtgtcggagagcaccctgtcccggctggagagcgggcagcgccgtgcgaccctggagctgctgctgccgctcgcccggatctacgacgtccccctggacgacctcgtcggcgccccgcgcacgggcgacccccgcatccacctgaagccggtcaggcgcttcgggatggtcttcgtgccgctgtcccggcggccgggcggcacccaggccttcaaaatgatcatcccgagccgtccggcgccgctcgaaccgaccccgcagacccacgaggggtccgagtggctgtacgtgctcagcggccgtctgcggttgctggtcggcgagcgcgacctgacgctgtcgcccggtgaggcggccgagttcgacacgtcgctgccgcactggctgggcagcgccgacggcggcgcggtcgaactcctcgtcctgttcgggctgcagggcgtgcgggcccatgtgcacagcggctgagagcttcctgcccgacggcgtcgccgagcgggtcggctgggcgcgcgaggcggccgaggcgacgccggaccggtcggcggagggcccgcgcgacagtcctgagggggcgtcgcgtccgcgtgttgcccggcagcccgcccggtccgtcgcccggcgtcacatccgtgcgtcgcccggcagcccgcccggtccgtcatccggcgtcacgcccggtccgtcgcccggcgtcacgcccggtccgtcatccggcgtcacgcccggtccgtcacccggcggcaggcctccacgtacccgcgcaccagtgcccgcccctcgtcctcgcggcgccgggccagggcgtagcggctgggggacaggccgcggaccgggcgggtgaccaccccgcccagggtgatcagcggggcgttgcccgtggccaccaggcagatgccgagcccggcgaccagggcctcgtacgtctcctccgtgccggagatctcggcgccgacgcgcggcggacgggcggcggggccgtcgagtgcgcgccgttcgtccagcgccagccagaagtcgcgcaggacgcccgcctccgggggcagggcgaggaacggctcgccggccaggtcggcgaagtcgatctcctcgcgggcggcgagggggtggctgtcggggagggcgaccaggcggggctcctcggcgaccaccgtccaggcgtagcggtcggcgtcgggcagcggcagccagacgtacgcgacgtcggccgtgccgtcggccaggcccgcggtcgggtcctcccagctcatctgccgcagctgcaggaccgcctccgggtgggccgcggtgaagcgggagcggatcgccgggagcagcccgccgcggccggggctggtgctcatgccgacgacgagggtgtcgcgccgggccgcacgggccgcctccaccgccgccgcgccctcggtccagtcggccagcatccgccgggcgtgcggcagcagggccgtgcccgcctcggtgagggtcacgccccgggggccgcggtggaacagctcggcgcccaactgccgttccagggcccggatctgcttgctcagcgcgggctgtgacacgtacaggagttcggccgcccgcgtgaagtgcagctcctcggccaccgtcgcgaagtagcgcagctcccgcacatgtacgtccgtcgtcatgcccatgggttatcaccgcgggtcttggaccggcaaccggcttgtggacgagggtggttggcgtcggaacaaggcgacagaggaaaccgagggagtcgggatgaacaaggtgtggctgatcaccggggcgagcagcggcttcgggcgggcgatcgccgaggcggccctggccgacggcgacgtcgtggtcggcgcggctcggcgccccgaggcgctggacgacctcgtggccgcgcacccggaccagatggaggcgctgcgcctggacgtcgccgacacggccgccgccggggacgccgtacgggacgtggtggcgcggcacggcagggtggacgtattggtcaacaacgcgggccgcacacacgtcggtgccctcgaggagaccggcgaggacgaactgcgggcgctgttcgacgtgcacgtcttcggcccggccgcgctgacgcgcgcggtactgccgtccatgcgggagcggcgttcgggcgcgatcgtgcagatgagcagcatgggcgggcagatgtccttcgcgggcttctccgcgtacagcggcacgaagttcgccctggagggcatgtccgaggggctcgcggacgaggtccgggacttcggcatcaaggtgctgatcgtcgagccgggctccttccgcaccggcctgttcgaggccgggaacgccgggatcagcgccgacagcggcgtgtacgccaaggtcggcgagacccgcgggatgatcgccgcgggcgacggcagccagcccggcgaccccgccagggcggccgcggtcatccgcgcggccctcgcggccgagcacactccgctgcgcctgccgctgggcgacgacggcgtcaccgcggtcctcggccacctcgaccgggtccgcgaggaggtcgagacctgggagaagcagacccgggccacggcgttcgacgactgaggggcagcggggtgtcggttcggcaccttcggtgcccgcacccgaccgcacccgactgtgcccgactgcacccgaccgtgcccgatcgtgcccgtgcccatgcccatgcccatgcccatgcccatgcccatgcccatgcccgtgcccgtgcccgcgtccgtgccgaaccaggagtccgccgtgctctcgtccctgaaggccgtcaacctgctggtgatgttcctgctggaactcgcggtgtacacggcggtcgtgctctggggggtcgccgtcggcggcacatggccggtcgaggtggccctgggggtgggcgcgccggtcgtgatgatggcggcgtgggcgctgttcgggtcgccgcgcgcccgccgtccggcgcgcggggccgggcggttcgtcctggaggtgctctggttcggtgccggtgcggccgccctggccgcctccgggagaccgtggtgggcggccgccctcgccggggtctgcctggtcaacgcggtgctcagacggttgtggaagcagtgacgcccggcgcgcccgcgacccgcgcaccgccccccgcgcggaccgcgcttacgatgcgcgaggccgcacccgtcgccgcaccaccctctcgaacaggagcacggtactcgtgtcgataccgccaccgccggggccccaagggcagtacccccagggtccgtacgctccgcagtgggggcaccccctcgcgccgtacccccggccggctcccgtgagcgggctcgccgtcgccgcgttcgtcctcggcgtcctgtgcttcctgccggcggtcggactggtcctcgggctggtcgcgctggcccggatccgcaggcggggcgaacgcggcaaggggttcgcggtggccggctgcgtgctgtcctccgtggggctggccctgtggacgctgacgctgtcgacgggcgccgcgggcgacttctgggacggcttccgggacgccgcgcgcggcgggggcaccgcctactccctggagaagggccagtgcttcaccacccccagcggctccctccaaggggtgacgtacgacgtcgacgaggtgccctgcgcgcgggagcacgacggcgaggtcttcgcctccttcgacctgccggacggttcctacccgggcgacggggagatcacgcgggccgccgacgaccggtgctacgccctccaggacgcctacgcgatggaccggtgggcactgccgaccgacgtcgacgtgtactacctgaccccgaccgccgcgagctggcggaccggcgaccgcgagatcacctgcctgttcggcaacacggacgagcggggcacgctgaccggctcgctgcgcaacgacggcgcgcggttcgacgcggaccagcacacctacctgctcgcggagggctacctgaaccgggccatggacgaggtgcccgcggcggaggcggtcgaggacgacctcgcgggctaccggacctgggccgggcaggtctcggaggcgctcaggggcgaggtcgcgatgctggacgggcacgagtggcccgccggcgccgagcgcccggtcgccgcgctgaccgacgacctgcggtcggcgcaggaggagtggggcctggcggctaaggccgccgacctcgacgcgtactacgagcactacggcaagggctacgacctcgtcgtcgccgacagcacggtcaccgcacgcaaggctctgggcctggccaccacgccgccggactacgagggcggcgagggcgggggagacgaccccggcgtggaggtgtgacagcggccatagcggggagaaagtgcctgcgtaaagccctcgggcggcgcaagtcatcacatcgagtgattctttggcctttgcttgcctgggccaacctacggttgccacgctgttgctgtctgtacaacctgatgggagcggccagtgacattcggtgagcagccggcgtatctgcgtgtcgcgggtgatctccgcaagaagatcgccgacggcctgctgccgccccatacccgcctcccgtcccaggcgcggatccgcgaggagtacggggtctcggacaccgtcgccctggaggcccgcaaggtgctgatggccgagggcctggtcgagggccgctccggttccggcacctacgtgcgcgagcggcccgtcccgcggcgcgtcgcccgctccggataccggccggccggcggggccacgcccttccgccaggagcaggccgacggggacgcgcgcggcacctgggagtcgcgcagcgagcaggccgaggcgagcggtgccgtggccgagcggctcgggatcaagcccggtgaccgggtgatgtgcacgcggtacgtcttccgggaggccggtgaggccgtcatgctctccacctcctgggagccgctggacctgaccggccgcaccccggtgatgctgcccgaggaagggccgctcggcgggatgggtgtcgtggagcggatggccgccatcgacgtcgtcgtcgacaacgtcaccgaggaggtcggcgcccgtcccggcctcgccgaggagttgctcgccctgggcggcgttccgggacacgtggtgctggtcgtccagcgcacgttctacgcctcggggcgtgccgtggagaccgccgacgtggtcgtcccggccgaccgctaccgggtggcgtaccacctgcccgtcaggtagcccgtcgggcagcccctcaagcagggccgtggccgggagtgttcgggggctctgccgcgatgcggggcggcggggtgagacggcggggcgggacggcggtgtgagatggcgcacgccagtcgtgcgcctcccgtgtcccgttcccccgctcacgcatccgccggggcccgcggcgtcgttcgcccggcgccggaatccggtcgttcccccaggtcgcttccccggtgcccggcacgcctgtgaccggaggcatcggtgtgcggagacggcgcgttccgcgtcgtgcgccccctgcgttctggctggttgcgtacctctttgtgcaaagccgtgttcgctccgtgaaggttgggcgtaggctcgggcatatgcggattgcggtttccttggcgggcggggcgcggcg

SEQ ID NO: 40 - DNA, 1131 bp, synthetic construct
  source 1..1131: mol_type = other DNA
  misc_feature 1..1131: note = outer region of 5' side of Actinorhodin biosynthetic gene cluster
atccactccagtacgcgtacgggtgggctgtcctcgggtgccggcaggaggccgcgggccctctcgaacacggcggtcacctgccggccgccctcccgcaccagcccggacagcgcgcgcagggcccgggcggggtccgcgtgcggggtcgggtcgtccgccggggcggtggcccacagcggtacctcgacgatcgccgtggcaccgccgtaccgctggggcgcgcaccaggtggacaggccgatgtcctcggacccggccgccggccgcgcggtgctgcccggcggcggcaggacatggatgccgggggccggattctcccagtacagggcgtcgtacgtgccgtgctggaccgggacccccagggcggcggcggacgccgcgaagggggcggcgagtccggggaggtcgcgggtcagctgggcccaggtgccgcccgcgtcgacgttgtgcagggagcactggaggacggggcgcaggtcgtcgatcacgtcgaacagggcacggctctccgggagtggccggccgacgatcggggcccactccggctgctccgcggcgaccgggcggaaggcggcacggtagtacgacgccagggacggggcggggccggccgtcgcggtctcgatgccctcgctcagcgcggcgccgtccgggtcgaggcacaggacgatgtcccaggtgacggcctcggggtcggtcgccggggagcgccggtcgccgcctgcgaccagctccgccagcgccagtgccgtcgcgccgcccaccggctcgtccgggtgcggccgggccaccaccaggacgtgccggggtccgtggcccaccgacagcatcaggagcggccggcccgcccgggacgtgccgacacgacacaggcggccggtgcccgggaaacgggagaccagccgtcgcgccgactcggtgacctccgcgaccgtggggtatcggttcatcgggcgtgtccggtcaggctccgccgttgccgctctcgtccgccatgccgtctccttccgacggtgcccgtgggtacccgtgggtacctgtgctgcttttcgcgcctgtgctgcctgtggtgtgcgaggcgcgtcgtgccgctgtcagcgtccgttcaccggatcaccgctgtcaatg

SEQ ID NO: 41 - DNA, 1083 bp, synthetic construct
  source 1..1083: mol_type = other DNA
  misc_feature 1..1083: note = outer region of 3' side of Actinorhodin biosynthetic gene cluster
gatcagctcgcggaggatgtcggcgtggccggcgtggcggccggtctcctccaccatgtgggtgagggcccagcggacactgggcgcggggcggcccggtcgcggccgggggagcggtgcgccgaggtcggtgcaggcgtcgagcacgcggttcgcccgttcgacggcctcccggtagcgggcgacgacgtcggcgacgccgtcctgggacgcggcccggaacgtcgccggccagcttcgcacctcctccccgaggaagaccgcgcgctcgacgtgggtcaggtggttgagcagcccgagcaggttggtgccggacgccaccgccgccgtgcggacctgcggttcgggggcgtcctcgaccttgccggcgatcgaggtccgcaggtagtcgaggaacccgcgcagggtctcggcctcaccgccgccggttcggggcggcggggtgtcccggcggtgggtgcggggggtggtgggcatggtgaccggcctccggaaggtgtggggcgggcgggccgcgggcgcggggcccgtcagtccgcgcggcggacgagcaggacgtggtcgacgacctcggcggtgcgcccgcccgggccggtcgcggtccggcgtggcgcctcggcccgttcgacccgccacgtcgccgggtccagggcgaggtccgccgcgacctcctgcggggccgggtggcgcgcgtcggggtcctggtcccacgaccacggcgccgtcgagccgtggtcgacgaccagcagccgcccgcccgggcgcagcgcgtgcgcggccccgcgcaggaccgacgcgcggtccaggtcgaagggcgtgtggaggtagtgcgcgctgaccaggtcgaaccggccctcggggaaggagtcgcgcaggtcgtgccgcacggcgtcgaccaggtcgccgaggccgtgggtccgtgcgtgccccgcgagccgctcggccgcgaccccggagatgtccacggccgtgacccgccagccccgccgggcaagccacagcgcgtcgccgccgctgccgcaccccaggtccagggcgtcgccgggcggcaggccggtgaccgtctcgaccaggcggacgttc

SEQ ID NO: 42 - DNA, 45 bp, synthetic construct
  source 1..45: mol_type = other DNA
  misc_feature 1..45: note = sco5071-5092del-left-F
agctatgaccatgattacgaattcatccactccagtacgcgtacg

SEQ ID NO: 43 - DNA, 34 bp, synthetic construct
  source 1..34: mol_type = other DNA
  misc_feature 1..34: note = sco5071-5092del-left-R
cgcgagctgatccattgacagcggtgatccggtg

SEQ ID NO: 44 - DNA, 34 bp, synthetic construct
  source 1..34: mol_type = other DNA
  misc_feature 1..34: note = sco5071-5092del-right-F
ccgctgtcaatggatcagctcgcggaggatgtcg

SEQ ID NO: 45 - DNA, 45 bp, synthetic construct
  source 1..45: mol_type = other DNA
  misc_feature 1..45: note = sco5092del-rightR
tcgaataagcttgcatgcctgcaggaacgtccgcctggtcgagac

SEQ ID NO: 46 - DNA, 7560 bp, synthetic construct
  source 1..7560: mol_type = other DNA
  misc_feature 1..7560: note = pPacI-int-delta act
atctcatgaccaaaatcccttaattaagtgcgtcgggtgatgctgccaacttactgatttagtgtatgatggtgtttttgaggtgctccagtggcttctgtttctatcagctgtccctcctgttcagctactgacggggtggtgcgtaacggcaaaagcaccgccggacatcagcgctagcggagtgtatactggcttactatgttggcactgatgagggtgtcagtgaagtgcttcatgtggcaggagaaaaaaggctgcaccggtgcgtcagcagaatatgtgatacaggatatattccgcttcctcgctcactgactcgctacgctcggtcgttcgactgcggcgagcggaaatggcttacgaacggggcggagatttcctggaagatgccaggaagatacttaacagggaagtgagagggccgcggcaaagccgtttttccataggctccgcccccctgacaagcatcacgaaatctgacgctcaaatcagtggtggcgaaacccgacaggactataaagataccaggcgtttccccctggcggctccctcgtgcgctctcctgttcctgcctttcggtttaccggtgtcattccgctgttatggccgcgtttgtctcattccacgcctgacactcagttccgggtaggcagttcgctccaagctggactgtatgcacgaaccccccgttcagtccgaccgctgcgccttatccggtaactatcgtcttgagtccaacccggaaagacatgcaaaagcaccactggcagcagccactggtaattgatttagaggagttagtcttgaagtcatgcgccggttaaggctaaactgaaaggacaagttttggtgactgcgctcctccaagccagttacctcggttcaaagagttggtagctcagagaaccttcgaaaaaccgccctgcaaggcggttttttcgttttcagagcaagagattacgcgcagaccaaaacgatctcaagaagatcatcttattaatcagataaaatatttctagatttcagtgcaatttatctcttcaaatgtagcacctgaagtcagccccatacgatataagttgtaattctcatgtttgacagcttatcatcgataagctttaatgcggtagtttatcacagttaaattaatgtgagttagctcactcattaggcaccccaggctttacactttatgcttccggctcgtatgttgtgtggaattgtgagcggataacaatttcacacaggaaacagctatgaccatgattacgaattcatccactccagtacgcgtacgggtgggctgtcctcgggtgccggcaggaggccgcgggccctctcgaacacggcggtcacctgccggccgccctcccgcaccagcccggacagcgcgcgcagggcccgggcggggtccgcgtgcggggtcgggtcgtccgccggggcggtggcccacagcggtacctcgacgatcgccgtggcaccgccgtaccgctggggcgcgcaccaggtggacaggccgatgtcctcggacccggccgccggccgcgcggtgctgcccggcggcggcaggacatggatgccgggggccggattctcccagtacagggcgtcgtacgtgccgtgctggaccgggacccccagggcggcggcggacgccgcgaagggggcggcgagtccggggaggtcgcgggtcagctgggcccaggtgccgcccgcgtcgacgttgtgcagggagcactggaggacggggcgcaggtcgtcgatcacgtcgaacagggcacggctctccgggagtggccggccgacgatcggggcccactccggctgctccgcggcgaccgggcggaaggcggcacggtagtacgacgccagggacggggcggggccggccgtcgcggtctcgatgccctcgctcagcgcggcgccgtccgggtcgaggcacaggacgatgtcccaggtgacggcctcggggtcggtcgccggggagcgccggtcgccgcctgcgaccagctccgccagcgccagtgccgtcgcgccgcccaccggctcgtccgggtgcggccgggccaccaccaggacgtgccggggtccgtggcccaccgacagcatcaggagcggccggcccgcccgggacgtgccgacacgacacaggcggccggtgcccgggaaacgggagaccagccgtcgcgccgactcggtgacctccgcgaccgtggggtatcggttcatcgggcgtgtccggtcaggctccgccgttgccgctctcgtccgccatgccgtctccttccgacggtgcccgtgggtacccgtgggtacctgtgctgcttttcgcgcctgtgctgcctgtggtgtgcgaggcgcgtcgtgccgctgtcagcgtccgttcaccggatcaccgctgtcaatggatcagctcgcggaggatgtcggcgtggccggcgtggcggccggtctcctccaccatgtgggtgagggcccagcggacactgggcgcggggcggcccggtcgcggccgggggagcggtgcgccgaggtcggtgcaggcgtcgagcacgcggttcgcccgttcgacggcctcccggtagcgggcgacgacgtcggcgacgccgtcctgggacgcggcccggaacgtcgccggccagcttcgcacctcctccccgaggaagaccgcgcgctcgacgtgggtcaggtggttgagcagcccgagcaggttggtgccggacgccaccgccgccgtgcggacctgcggttcgggggcgtcctcgaccttgccggcgatcgaggtccgcaggtagtcgaggaacccgcgcagggtctcggcctcaccgccgccggttcggggcggcggggtgtcccggcggtgggtgcggggggtggtgggcatggtgaccggcctccggaaggtgtggggcgggcgggccgcgggcgcggggcccgtcagtccgcgcggcggacgagcaggacgtggtcgacgacctcggcggtgcgcccgcccgggccggtcgcggtccggcgtggcgcctcggcccgttcgacccgccacgtcgccgggtccagggcgaggtccgccgcgacctcctgcggggccgggtggcgcgcgtcggggtcctggtcccacgaccacggcgccgtcgagccgtggtcgacgaccagcagccgcccgcccgggcgcagcgcgtgcgcggccccgcgcaggaccgacgcgcggtccaggtcgaagggcgtgtggaggtagtgcgcgctgaccaggtcgaaccggccctcggggaaggagtcgcgcaggtcgtgccgcacggcgtcgaccaggtcgccgaggccgtgggtccgtgcgtgccccgcgagccgctcggccgcgaccccggagatgtccacggccgtgacccgccagccccgccgggcaagccacagcgcgtcgccgccgctgccgcaccccaggtccagggcgtcgccgggcggcaggccggtgaccgtctcgaccaggcggacgttcctgcaggcatgcaagcttattcgatatcatgtcggaccggagttcgaggtacgcggcttgcaggtccaggaaggggacgtccatgcgagtgtccgttcgagtggcggcttgcgcccgatgctagtcgcggttgatcggcgatcgcaggtgcacgcggtcgatcttgacggctggcgagaggtgcggggaggatctgaccgacgcggtccacacgtggcaccgcgatgctgttgtgggcacaatcgtgccggttggtaggatcctcgaggacaggaggctgccatatgccgaacaacgcgcttcagacgatcatcaacgcccgcctgcccggtgaggaaggcctgtggcaaatccacctgcaagacggcaagatctcggccatcgacgcccagtccggagtgatgccgatcacggagaacagcctggacgcggagcagggcctggtgatccccccgttcgtcgagccccacatccacttggacaccacccagacggccggccagcccaactggaaccagtcgggcaccctgttcgagggcatcgagcggtgggccgagcgcaaggcgctgctgacccacgacgacgtgaagcagcgggcgtggcagaccctcaagtggcagatcgccaacggcatccagcacgtacgcacgcacgtggacgtctccgatgcgaccctcacggccctgaaggccatgctcgaagtcaagcaggaggtggccccgtggatcgacctccagatcgtcgccttcccgcaggagggcatcctctcgtaccccaacggcgaagccctcctggaggaggccctgcggctgggagccgacgtcgtcggtgccatcccgcacttcgagttcacccgcgagtacggcgttgagagcctgcacaagaccttcgcgctggcgcagaagtacgaccgcctgatcgacgtccactgcgacgagatcgacgacgagcagtcccggttcgtggagaccgtcgcggcactggcccatcacgagggcatgggtgcccgcgtcacagcgtcccacaccacggccatgcactcctacaacggcgcctacacctcccgcctgttccgcctcctgaagatgtcgggcatcaacttcgtcgccaatcccctcgtgaacatccacctccagggcaggttcgacacgtacccgaaacggcggggcattacccgcgtcaaggagatgctcgaatcggggatcaacgtgtgcttcgggcacgcggacgtcttcgacccgtggtacccgctcggcaccgccaacatgctccaggtcctgcacatgggcctgcacgtctgccagctgatgggctacgggcagatcaacgacgggctgaacctcatcacgcaccacagtgcccgtaccctgaacctccaggactacggcatcgccgctgggaactccgccaacctgatcatcctgccagcggagaacggcttcgacgcgctccgtcggcaggtgccggtgcgctacagcgtccgaggcggcaaggtcatcgcgagcacccagcccgcacagaccaccgtctatctggagcagccggaggcgatcgactacaagcgctgatctagagtcggctagcttcacgctgccgcaagcactcagggcgcaagggctgctaaaggaagcggaacacgtagaaagccagtccgcagaaacggtgctgaccccggatgaatgtcagctactgggctatctggacaagggaaaacgcaagcgcaaagagaaagcaggtagcttgcagtgggcttacatggcgatagctagactgggcggttttatggacagcaagcgaaccggaattgccagctggggcgccctctggtaaggttgggaagccctgcaaagtaaactggatggctttcttgccgccaaggatctgatggcgcaggggatcaagatctgatcaagagacaggatgaggatcgtttcgcatgattgaacaagatggattgcacgcaggttctccggccgcttgggtggagaggctattcggctatgactgggcacaacagacaatcggctgctctgatgccgccgtgttccggctgtcagcgcaggggcgcccggttctttttgtcaagaccgacctgtccggtgccctgaatgaactccaagacgaggcagcgcggctatcgtggctggccacgacgggcgttccttgcgcagctgtgctcgacgttgtcactgaagcgggaagggactggctgctattgggcgaagtgccggggcaggatctcctgtcatctcaccttgctcctgccgagaaagtatccatcatggctgatgcaatgcggcggctgcatacgcttgatccggctacctgcccattcgaccaccaagcgaaacatcgcatcgagcgagcacgtactcggatggaagccggtcttgtcgatcaggatgatctggacgaagagcatcaggggctcgcgccagccgaactgttcgccaggctcaaggcgcggatgcccgacggcgaggatctcgtcgtgacccatggcgatgcctgcttgccgaatatcatggtggaaaatggccgcttttctggattcatcgactgtggccggctgggtgtggcggaccgctatcaggacatagcgttggctacccgtgatattgctgaagagcttggcggcgaatgggctgaccgcttcctcgtgctttacggtatcgccgctcccgattcgcagcgcatcgccttctatcgccttcttgacgagttcttctgagcgggactctggggttcgaaatgaccgaccaagcgacgcccaacctgccatcacgagatttcgattccaccgccgccttctatgaaaggttgggcttcggaatcgttttccgggacgccctcgcggacgtgctcatagtccacgacgcccgtgattttgtagccctggccgacggccagcaggtaggccgacaggctcatgccggccgccgccgccttttcctcaatcgctcttcgttcgtctggaaggcagtacaccttgataggtgggctgcccttcctggttggcttggtttcatcagccatccgcttgccctcatctgttacgccggcggtagccggccagcctcgcagagcaggattcccgttgagcaccgccaggtgcgaataagggacagtgaagaaggaacacccgctcgcgggtgggcctacttcacctatcctgccccgctgacgccgttggatacaccaaggaaagtctacacgaaccctttggcaaaatcctgtatatcgtgcgaaaaaggatggatataccgaaaaaatcgctataatgaccccgaagcagggttatgcagcggaaaagcgctgcttccctgctgttttgtggaatatctaccgactggaaacaggcaaatgcaggaaattactgaactgaggggacaggcgagagacgatgccaaagagctcctgaaaatctcgataactcaaaaaatacgcccggtagtgatcttatttcattatggtgaaagttggaacctcttacgtgccgatcaacgtctcattttcgccaaaagttggcccagggcttcccggtatcaacagggacaccaggatttatttattctgcgaagtgatcttccgtcacaggtatttattcggcgcaaagtgcgtcgggtgatgctgccaacttactgatttagtgtatgatggtgtttttgaggtgctccagtggcttctgtttctatcagctcctgaaaatctcgataactcaaaaaatacgcccggtagtgatcttatttcattatggtgaaagttggaacctcttacgtgccgatcaacgtctcattttcgccaaaagttggcccagggcttcccggtatcaacagggacaccaggatttatttattctgcgaagtgatcttccgtcacaggtatttattcggcgcaaagtgcgtcgggtgatgctgccaacttactgatttagtgtatgatggtgtttttgaggtgctccagtggcttctgtttctatcagggctggatgatcctccagcgcggggatctcatgctggagttcttcgcccaccccaaaaggatctaggtgaagatcctttttgata

SEQ ID NO: 47 - DNA, 45 bp, synthetic construct; identical to SEQ ID NO: 42
  source 1..45: mol_type = other DNA
  misc_feature 1..45: note = sco5071-5092del-left-F

SEQ ID NO: 48 - DNA, 45 bp, synthetic construct; identical to SEQ ID NO: 45
  source 1..45: mol_type = other DNA
  misc_feature 1..45: note = sco5092del-rightR

SEQ ID NO: 49 - DNA, 1150 bp, synthetic construct
  source 1..1150: mol_type = other DNA
  misc_feature 1..1150: note = center region of Actinorhodin biosynthetic gene cluster
ccgtcttcctgatcaatctgccgatcggcgtggccgtgatcgtcggcgcggtcctgctgctgcccgagggcaaggcgcccgtgcggccgaagttcgacgtcgtcggcatggcgctggtgacgtccgggctcaccctgctcatcttcccgctcgtccaggggcgcgaacgcggctggcccgcctgggcgttcgtgctgatgctggccggagcggccgtgctcgtcggcttcgtcgcccacgaactgcggcaggagaggcgcggcggcgccacgctcatcgagctcagcctgctgcgcaggtcccgctacgccgcgggactggcggtggcactggtgttcttcaccggcgtctccggaatgtcgctgctgctcgccctgcacctgcagatcggcctgggcttcagccccaccagggccgcgctgaccatgacgccctggtcggtgttcctcgtcgtcggcgcgatcctgaccggggcggtgctgggatcgaagttcggccgcaaggccctgcacggcgggctcgtggtgctggcgctgggcgtgctgatcatgctgttgacgatcggcgaccaggccggcgggctgaccagctgggagctcgtccccggtatcgccgttgccgggctcggcatgggcatcatgatcggactgctcttcgacatcgccctggccgacgtcgacaagcaggaggccggtaccgcctccggcgtcctcaccgcggtccagcagctcggcttcaccgtgggcgtcgcggtgctcgggaccctgttcttcgggctgctcggctcacaggccacggcgagcgtcgacgacggcgcgagccgggcccgcaccgaactcgccgccgccggggcgagcacgaccgagcaggaccggctcctggccgacctgcgggtgtgcctgcgggaatcggcgagtcagcaggactccgaacggacgccggacagctgccgaaacctccagcaggcccggccggcggtggccgaggccacggcgcgggcctggcggacggcccacaccgagaacttcagcaccgcgatggtccgcacgctctgggtggtgatcgcactgctggcggtctccttcgcgctggccttccggctgccgcccaagccgcgtgaggaagagggcttctgatgacacgcacactg

SEQ ID NO: 50 - DNA, 24 bp, synthetic construct
  source 1..24: mol_type = other DNA
  misc_feature 1..24: note = act-del-CK F
cggtccgtcttcctgatcaatctg

SEQ ID NO: 51 - DNA, 23 bp, synthetic construct
  source 1..23: mol_type = other DNA
  misc_feature 1..23: note = act-del-CK R
agcagtgtgcgtgtcatcagaag

SEQ ID NO: 52 - DNA, 22 bp, synthetic construct
  source 1..22: mol_type = other DNA
  misc_feature 1..22: note = act-del-seq F1
tgggtacctgtgctgcttttcg

SEQ ID NO: 53 - DNA, 21 bp, synthetic construct
  source 1..21: mol_type = other DNA
  misc_feature 1..21: note = act-del-seq R1
agctcgtcgggaagcagcttc

SEQ ID NO: 54 - DNA, 22 bp, synthetic construct
  source 1..22: mol_type = other DNA
  misc_feature 1..22: note = act-del-seq F2
gtccgtgcacgtcgaggagaag

SEQ ID NO: 55 - DNA, 21 bp, synthetic construct
  source 1..21: mol_type = other DNA
  misc_feature 1..21: note = act-del-seq R2
cactacctccacacgcccttc

SEQ ID NO: 56 - DNA, 534 bp, synthetic construct
  source 1..534: mol_type = other DNA
  misc_feature 1..534: note = actVB
atggcagccgaccagggaatgctccgggacgccatggcccgggtgccggccggggtggcgctcgtcaccgcccatgaccgcgggggagtcccgcacggtttcaccgccagttcgttcgtgtccgtctcgatggagccgccactggcactggtctgcctggctcgtacggccaactccttcccggtgttcgacagttgcggcgagttcgcggtgagcgtgctgcgcgaggaccacacggacctggccatgcgcttcgcgcgcaagtccgcggacaagttcgcgggcggggagttcgtccgtaccgcgcggggagcgaccgtgctcgacggagcggtcgcggtcgtcgagtgcacggtccacgagcgctacccggcgggcgaccacatcatcctgctcggcgaggtccagtccgtgcacgtcgaggagaagggcgtaccggcggtctacgtggaccgccggttcgccgccctgtgctcggcggcgggtgcctgcccgtccgccaccgggcggggcgtgcccgcgcatgccggctga

SEQ ID NO: 57 - DNA, 1002 bp, synthetic construct
  source 1..1002: mol_type = other DNA
  misc_feature 1..1002: note = outer region of 5' side of actVB
gcggacgcccgtacccatctgcgcgaggtgctcggtgccaacagccgggccacgctccgccacgcggcggccgccgccgggccggcgtcatgacggtcgaggtccgtgaggtcgccgagggtgtctacgcctacgagcaggcccccggcggctggtgcgtcagcaacgcgggcatcgtggtgggcggcgacggcgcgctcgtcgtcgacacgctgtcgacgatcccgagggcgcggcggctggcggagtgggtcgacaagctcgccgcgggccccggccgtaccgtggtcaacacccacttccacggcgaccacgccttcggcaaccaggtcttcgcgccggggacgcggatcatcgcgcacgaggacatgcggtccgccatggtgacgaccggcctggccctcaccgggctctggccgcgggtcgactggggcgagatcgagctgaggccgccgaacgtgaccttccgcgaccggttgaccctgcacgtcggcgagcgacaggtcgaactgatctgcgtcggccccgcgcacaccgatcacgacgtggtggtctggctgcccgaggagcgggtgctgttcgcgggggacgtcgtcatgtcgggcgtcactccgttcgccctcttcggttcggtggccggcacgctggccgcgctcgaccggctggcggagctggagcccgaggtggtcgtcggcgggcacggcccggtggcgggacccgaggtgatcgacgccaaccgggactatctgcgctgggtccagcgcctcgccgccgatgcggtcgaccgccggctgacaccgttgcaggccgcgcgccgggcggacctcggcgccttcgccgggctgctggacgcggagcgcctcgtcgcgaacctgcaccgggcccacgaggagctgctgggcgggcacgtgcgtgacgccatggcgatcttcgcggagctggtcgcctacaacggtgggcagctgcccacctgcctcgcctagggagttcgaagatggcagc

SEQ ID NO: 58 - DNA, 1083 bp, synthetic construct; identical to SEQ ID NO: 41
  source 1..1083: mol_type = other DNA
  misc_feature 1..1083: note = outer region of 3' side of actVB

SEQ ID NO: 59 - DNA, 45 bp, synthetic construct
  source 1..45: mol_type = other DNA
  misc_feature 1..45: note = sco5092del-leftF
agctatgaccatgattacgaattcgcggacgcccgtacccatcgt

SEQ ID NO: 60 - DNA, 33 bp, synthetic construct
  source 1..33: mol_type = other DNA
  misc_feature 1..33: note = sco5092del-lefrR
cgagctgatcgctgccatcttcgaactccctag

SEQ ID NO: 61 - DNA, 31 bp, synthetic construct
  source 1..31: mol_type = other DNA
  misc_feature 1..31: note = sco5092del-rightF
agatggcagcgatcagctcgcggaggatgct

SEQ ID NO: 62 - DNA, 45 bp, synthetic construct; identical to SEQ ID NO: 45
  source 1..45: mol_type = other DNA
  misc_feature 1..45: note = sco5092del-rightR

SEQ ID NO: 63 - DNA, 7431 bp, synthetic construct
  source 1..7431: mol_type = other DNA
  misc_feature 1..7431: note = pPacI-int-delta actVB
atctcatgaccaaaatcccttaattaagtgcgtcgggtgatgctgccaacttactgatttagtgtatgatggtgtttttgaggtgctccagtggcttctgtttctatcagctgtccctcctgttcagctactgacggggtggtgcgtaacggcaaaagcaccgccggacatcagcgctagcggagtgtatactggcttactatgttggcactgatgagggtgtcagtgaagtgcttcatgtggcaggagaaaaaaggctgcaccggtgcgtcagcagaatatgtgatacaggatatattccgcttcctcgctcactgactcgctacgctcggtcgttcgactgcggcgagcggaaatggcttacgaacggggcggagatttcctggaagatgccaggaagatacttaacagggaagtgagagggccgcggcaaagccgtttttccataggctccgcccccctgacaagcatcacgaaatctgacgctcaaatcagtggtggcgaaacccgacaggactataaagataccaggcgtttccccctggcggctccctcgtgcgctctcctgttcctgcctttcggtttaccggtgtcattccgctgttatggccgcgtttgtctcattccacgcctgacactcagttccgggtaggcagttcgctccaagctggactgtatgcacgaaccccccgttcagtccgaccgctgcgccttatccggtaactatcgtcttgagtccaacccggaaagacatgcaaaagcaccactggcagcagccactggtaattgatttagaggagttagtcttgaagtcatgcgccggttaaggctaaactgaaaggacaagttttggtgactgcgctcctccaagccagttacctcggttcaaagagttggtagctcagagaaccttcgaaaaaccgccctgcaaggcggttttttcgttttcagagcaagagattacgcgcagaccaaaacgatctcaagaagatcatcttattaatcagataaaatatttctagatttcagtgcaatttatctcttcaaatgtagcacctgaagtcagccccatacgatataagttgtaattctcatgtttgacagcttatcatcgataagctttaatgcggtagtttatcacagttaaattaatgtgagttagctcactcattaggcaccccaggctttacactttatgcttccggctcgtatgttgtgtggaattgtgagcggataacaatttcacacaggaaacagctatgaccatgattacgaattcgcggacgcccgtacccatctgcgcgaggtgctcggtgccaacagccgggccacgctccgccacgcggcggccgccgccgggccggcgtcatgacggtcgaggtccgtgaggtcgccgagggtgtctacgcctacgagcaggcccccggcggctggtgcgtcagcaacgcgggcatcgtggtgggcggcgacggcgcgctcgtcgtcgacacgctgtcgacgatcccgagggcgcggcggctggcggagtgggtcgacaagctcgccgcgggccccggccgtaccgtggtcaacacccacttccacggcgaccacgccttcggcaaccaggtcttcgcgccggggacgcggatcatcgcgcacgaggacatgcggtccgccatggtgacgaccggcctggccctcaccgggctctggccgcgggtcgactggggcgagatcgagctgaggccgccgaacgtgaccttccgcgaccggttgaccctgcacgtcggcgagcgacaggtcgaactgatctgcgtcggccccgcgcacaccgatcacgacgtggtggtctggctgcccgaggagcgggtgctgttcgcgggggacgtcgtcatgtcgggcgtcactccgttcgccctcttcggttcggtggccggcacgctggccgcgctcgaccggctggcggagctggagcccgaggtggtcgtcggcgggcacggcccggtggcgggacccgaggtgatcgacgccaaccgggactatctgcgctgggtccagcgcctcgccgccgatgcggtcgaccgccggctgacaccgttgcaggccgcgcgccgggcggacctcggcgccttcgccgggctgctggacgcggagcgcctcgtcgcgaacctgcaccgggcccacgaggagctgctgggcgggcacgtgcgtgacgccatggcgatcttcgcggagctggtcgcctacaacggtgggcagctgcccacctgcctcgcctagggagttcgaagatggcagcgatcagctcgcggaggatgtcggcgtggccggcgtggcggccggtctcctccaccatgtgggtgagggcccagcggacactgggcgcggggcggcccggtcgcggccgggggagcggtgcgccgaggtcggtgcaggcgtcgagcacgcggttcgcccgttcgacggcctcccggtagcgggcgacgacgtcggcgacgccgtcctgggacgcggcccggaacgtcgccggccagcttcgcacctcctccccgaggaagaccgcgcgctcgacgtgggtcaggtggttgagcagcccgagcaggttggtgccggacgccaccgccgccgtgcggacctgcggttcgggggcgtcctcgaccttgccggcgatcgaggtccgcaggtagtcgaggaacccgcgcagggtctcggcctcaccgccgccggttcggggcggcggggtgtcccggcggtgggtgcggggggtggtgggcatggtgaccggcctccggaaggtgtggggcgggcgggccgcgggcgcggggcccgtcagtccgcgcggcggacgagcaggacgtggtcgacgacctcggcggtgcgcccgcccgggccggtcgcggtccggcgtggcgcctcggcccgttcgacccgccacgtcgccgggtccagggcgaggtccgccgcgacctcctgcggggccgggtggcgcgcgtcggggtcctggtcccacgaccacggcgccgtcgagccgtggtcgacgaccagcagccgcccgcccgggcgcagcgcgtgcgcggccccgcgcaggaccgacgcgcggtccaggtcgaagggcgtgtggaggtagtgcgcgctgaccaggtcgaaccggccctcggggaaggagtcgcgcaggtcgtgccgcacggcgtcgaccaggtcgccgaggccgtgggtccgtgcgtgccccgcgagccgctcggccgcgaccccggagatgtccacggccgtgacccgccagccccgccgggcaagccacagcgcgtcgccgccgctgccgcaccccaggtccagggcgtcgccgggcggcaggccggtgaccgtctcgaccaggcggacgttcctgcaggcatgcaagcttattcgatatcatgtcggaccggagttcgaggtacgcggcttgcaggtccaggaaggggacgtccatgcgagtgtccgttcgagtggcggcttgcgcccgatgctagtcgcggttgatcggcgatcgcaggtgcacgcggtcgatcttgacggctggcgagaggtgcggggaggatctgaccgacgcggtccacacgtggcaccgcgatgctgttgtgggcacaatcgtgccggttggtaggatcctcgaggacaggaggctgccatatgccgaacaacgcgcttcagacgatcatcaacgcccgcctgcccggtgaggaaggcctgtggcaaatccacctgcaagacggcaagatctcggccatcgacgcccagtccggagtgatgccgatcacggagaacagcctggacgcggagcagggcctggtgatccccccgttcgtcgagccccacatccacttggacaccacccagacggccggccagcccaactggaaccagtcgggcaccctgttcgagggcatcgagcggtgggccgagcgcaaggcgctgctgacccacgacgacgtgaagcagcgggcgtggcagaccctcaagtggcagatcgccaacggcatccagcacgtacgcacgcacgtggacgtctccgatgcgaccctcacggccctgaaggccatgctcgaagtcaagcaggaggtggccccgtggatcgacctccagatcgtcgccttcccgcaggagggcatcctctcgtaccccaacggcgaagccctcctggaggaggccctgcggctgggagccgacgtcgtcggtgccatcccgcacttcgagttcacccgcgagtacggcgttgagagcctgcacaagaccttcgcgctggcgcagaagtacgaccgcctgatcgacgtccactgcgacgagatcgacgacgagcagtcccggttcgtggagaccgtcgcggcactggcccatcacgagggcatgggtgcccgcgtcacagcgtcccacaccacggccatgcactcctacaacggcgcctacacctcccgcctgttccgcctcctgaagatgtcgggcatcaacttcgtcgccaatcccctcgtgaacatccacctccagggcaggttcgacacgtacccgaaacggcggggcattacccgcgtcaaggagatgctcgaatcggggatcaacgtgtgcttcgggcacgcggacgtcttcgacccgtggtacccgctcggcaccgccaacatgctccaggtcctgcacatgggcctgcacgtctgccagctgatgggctacgggcagatcaacgacgggctgaacctcatcacgcaccacagtgcccgtaccctgaacctccaggactacggcatcgccgctgggaactccgccaacctgatcatcctgccagcggagaacggcttcgacgcgctccgtcggcaggtgccggtgcgctacagcgtccgaggcggcaaggtcatcgcgagcacccagcccgcacagaccaccgtctatctggagcagccggaggcgatcgactacaagcgctgatctagagtcggctagcttcacgctgccgcaagcactcagggcgcaagggctgctaaaggaagcggaacacgtagaaagccagtccgcagaaacggtgctgaccccggatgaatgtcagctactgggctatctggacaagggaaaacgcaagcgcaaagagaaagcaggtagcttgcagtgggcttacatggcgatagctagactgggcggttttatggacagcaagcgaaccggaattgccagctggggcgccctctggtaaggttgggaagccctgcaaagtaaactggatggctttcttgccgccaaggatctgatggcgcaggggatcaagatctgatcaagagacaggatgaggatcgtttcgcatgattgaacaagatggattgcacgcaggttctccggccgcttgggtggagaggctattcggctatgactgggcacaacagacaatcggctgctctgatgccgccgtgttccggctgtcagcgcaggggcgcccggttctttttgtcaagaccgacctgtccggtgccctgaatgaactccaagacgaggcagcgcggctatcgtggctggccacgacgggcgttccttgcgcagctgtgctcgacgttgtcactgaagcgggaagggactggctgctattgggcgaagtgccggggcaggatctcctgtcatctcaccttgctcctgccgagaaagtatccatcatggctgatgcaatgcggcggctgcatacgcttgatccggctacctgcccattcgaccaccaagcgaaacatcgcatcgagcgagcacgtactcggatggaagccggtcttgtcgatcaggatgatctggacgaagagcatcaggggctcgcgccagccgaactgttcgccaggctcaaggcgcggatgcccgacggcgaggatctcgtcgtgacccatggcgatgcctgcttgccgaatatcatggtggaaaatggccgcttttctggattcatcgactgtggccggctgggtgtggcggaccgctatcaggacatagcgttggctacccgtgatattgctgaagagcttggcggcgaatgggctgaccgcttcctcgtgctttacggtatcgccgctcccgattcgcagcgcatcgccttctatcgccttcttgacgagttcttctgagcgggactctggggttcgaaatgaccgaccaagcgacgcccaacctgccatcacgagatttcgattccaccgccgccttctatgaaaggttgggcttcggaatcgttttccgggacgccctcgcggacgtgctcatagtccacgacgcccgtgattttgtagccctggccgacggccagcaggtaggccgacaggctcatgccggccgccgccgccttttcctcaatcgctcttcgttcgtctggaaggcagtacaccttgataggtgggctgcccttcctggttggcttggtttcatcagccatccgcttgccctcatctgttacgccggcggtagccggccagcctcgcagagcaggattcccgttgagcaccgccaggtgcgaataagggacagtgaagaaggaacacccgctcgcgggtgggcctacttcacctatcctgccccgctgacgccgttggatacaccaaggaaagtctacacgaaccctttggcaaaatcctgtatatcgtgcgaaaaaggatggatataccgaaaaaatcgctataatgaccccgaagcagggttatgcagcggaaaagcgctgcttccctgctgttttgtggaatatctaccgactggaaacaggcaaatgcaggaaattactgaactgaggggacaggcgagagacgatgccaaagagctcctgaaaatctcgataactcaaaaaatacgcccggtagtgatcttatttcattatggtgaaagttggaacctcttacgtgccgatcaacgtctcattttcgccaaaagttggcccagggcttcccggtatcaacagggacaccaggatttatttattctgcgaagtgatcttccgtcacaggtatttattcggcgcaaagtgcgtcgggtgatgctgccaacttactgatttagtgtatgatggtgtttttgaggtgctccagtggcttctgtttctatcagctcctgaaaatctcgataactcaaaaaatacgcccggtagtgatcttatttcattatggtgaaagttggaacctcttacgtgccgatcaacgtctcattttcgccaaaagttggcccagggcttcccggtatcaacagggacaccaggatttatttattctgcgaagtgatcttccgtcacaggtatttattcggcgcaaagtgcgtcgggtgatgctgccaacttactgatttagtgtatgatggtgtttttgaggtgctccagtggcttctgtttctatcagggctggatgatcctccagcgcggggatctcatgctggagttcttcgcccaccccaaaaggatctaggtgaagatcctttttgata

SEQ ID NO: 64 - DNA, 21 bp, synthetic construct
  source 1..21: mol_type = other DNA
  misc_feature 1..21: note = sco5092del-seqF
tccgttcgccctcttcggttc

SEQ ID NO: 65 - DNA, 21 bp, synthetic construct
  source 1..21: mol_type = other DNA
  misc_feature 1..21: note = sco5092del-seqR
ctcaaccacctgacccacgtc

SEQ ID NO: 66 - DNA, 21 bp, synthetic construct
  source 1..21: mol_type = other DNA
  misc_feature 1..21: note = actVB-del-CK-F
tggaagaggtcctggggaaag

SEQ ID NO: 67 - DNA, 25 bp, synthetic construct
  source 1..25: mol_type = other DNA
  misc_feature 1..25: note = actVB-del-CK-R
aaacgactgaaggagttccgatgag

SEQ ID NO: 68 - DNA, 913 bp, synthetic construct
  source 1..913: mol_type = other DNA
  misc_feature 1..913: note = p15A ori
gcgctagcggagtgtatactggcttactatgttggcactgatgagggtgtcagtgaagtgcttcatgtggcaggagaaaaaaggctgcaccggtgcgtcagcagaatatgtgatacaggatatattccgcttcctcgctcactgactcgctacgctcggtcgttcgactgcggcgagcggaaatggcttacgaacggggcggagatttcctggaagatgccaggaagatacttaacagggaagtgagagggccgcggcaaagccgtttttccataggctccgcccccctgacaagcatcacgaaatctgacgctcaaatcagtggtggcgaaacccgacaggactataaagataccaggcgtttccccctggcggctccctcgtgcgctctcctgttcctgcctttcggtttaccggtgtcattccgctgttatggccgcgtttgtctcattccacgcctgacactcagttccgggtaggcagttcgctccaagctggactgtatgcacgaaccccccgttcagtccgaccgctgcgccttatccggtaactatcgtcttgagtccaacccggaaagacatgcaaaagcaccactggcagcagccactggtaattgatttagaggagttagtcttgaagtcatgcgccggttaaggctaaactgaaaggacaagttttggtgactgcgctcctccaagccagttacctcggttcaaagagttggtagctcagagaaccttcgaaaaaccgccctgcaaggcggttttttcgttttcagagcaagagattacgcgcagaccaaaacgatctcaagaagatcatcttattaatcagataaaatatttctagatttcagtgcaatttatctcttcaaatgtagcacctgaagtcagccccatacgatataagttgt

SEQ ID NO: 69 - protein, 427 aa, synthetic construct
  REGION 1..427: note = codA
MPNNALQTIINARLPGEEGLWQIHLQDGKISAIDAQSGVMPITENSLDAEQGLVIPPFVEPHIHLDTTQTAGQPNWNQSGTLFEGIERWAERKALLTHDDVKQRAWQTLKWQIANGIQHVRTHVDVSDATLTALKAMLEVKQEVAPWIDLQIVAFPQEGILSYPNGEALLEEALRLGADVVGAIPHFEFTREYGVESLHKTFALAQKYDRLIDVHCDEIDDEQSRFVETVAALAHHEGMGARVTASHTTAMHSYNGAYTSRLFRLLKMSGINFVANPLVNIHLQGRFDTYPKRRGITRVKEMLESGINVCFGHADVFDPWYPLGTANMLQVLHMGLHVCQLMGYGQINDGLNLITHHSARTLNLQDYGIAAGNSANLIILPAENGFDALRRQVPVRYSVRGGKVIASTQPAQTTVYLEQPEAIDYKR

SEQ ID NO: 70 - DNA, 1284 bp, synthetic construct
  source 1..1284: mol_type = other DNA
  misc_feature 1..1284: note = codAsm
atgccgaacaacgcgcttcagacgatcatcaacgcccgcctgcccggtgaggaaggcctgtggcaaatccacctgcaagacggcaagatctcggccatcgacgcccagtccggagtgatgccgatcacggagaacagcctggacgcggagcagggcctggtgatccccccgttcgtcgagccccacatccacttggacaccacccagacggccggccagcccaactggaaccagtcgggcaccctgttcgagggcatcgagcggtgggccgagcgcaaggcgctgctgacccacgacgacgtgaagcagcgggcgtggcagaccctcaagtggcagatcgccaacggcatccagcacgtacgcacgcacgtggacgtctccgatgcgaccctcacggccctgaaggccatgctcgaagtcaagcaggaggtggccccgtggatcgacctccagatcgtcgccttcccgcaggagggcatcctctcgtaccccaacggcgaagccctcctggaggaggccctgcggctgggagccgacgtcgtcggtgccatcccgcacttcgagttcacccgcgagtacggcgttgagagcctgcacaagaccttcgcgctggcgcagaagtacgaccgcctgatcgacgtccactgcgacgagatcgacgacgagcagtcccggttcgtggagaccgtcgcggcactggcccatcacgagggcatgggtgcccgcgtcacagcgtcccacaccacggccatgcactcctacaacggcgcctacacctcccgcctgttccgcctcctgaagatgtcgggcatcaacttcgtcgccaatcccctcgtgaacatccacctccagggcaggttcgacacgtacccgaaacggcggggcattacccgcgtcaaggagatgctcgaatcggggatcaacgtgtgcttcgggcacgcggacgtcttcgacccgtggtacccgctcggcaccgccaacatgctccaggtcctgcacatgggcctgcacgtctgccagctgatgggctacgggcagatcaacgacgggctgaacctcatcacgcaccacagtgcccgtaccctgaacctccaggactacggcatcgccgctgggaactccgccaacctgatcatcctgccagcggagaacggcttcgacgcgctccgtcggcaggtgccggtgcgctacagcgtccgaggcggcaaggtcatcgcgagcacccagcccgcacagaccaccgtctatctggagcagccggaggcgatcgactacaagcgctga

SEQ ID NO: 71 - DNA, 197 bp, synthetic construct
  source 1..197: mol_type = other DNA
  misc_feature 1..197: note = PermE
caggaaggggacgtccatgcgagtgtccgttcgagtggcggcttgcgcccgatgctagtcgcggttgatcggcgatcgcaggtgcacgcggtcgatcttgacggctggcgagaggtgcggggaggatctgaccgacgcggtccacacgtggcaccgcgatgctgttgtgggcacaatcgtgccggttggtaggatcc

SEQ ID NO: 72 - DNA, 115 bp, synthetic construct
  source 1..115: mol_type = other DNA
  misc_feature 1..115: note = PtipA
gggctgagggagccgacggcacgcggcggctcacggcgtggcacgcggaacgtccgggcttgcacctcacgtcacgtgaggaggcagcgtggacggcgtcagagaagggagcgga

SEQ ID NO: 73 - DNA, 589 bp, synthetic construct
  source 1..589: mol_type = other DNA
  misc_feature 1..589: note = pUC ori
ttgagatcctttttttctgcgcgtaatctgctgcttgcaaacaaaaaaaccaccgctaccagcggtggtttgtttgccggatcaagagctaccaactctttttccgaaggtaactggcttcagcagagcgcagataccaaatactgttcttctagtgtagccgtagttaggccaccacttcaagaactctgtagcaccgcctacatacctcgctctgctaatcctgttaccagtggctgctgccagtggcgataagtcgtgtcttaccgggttggactcaagacgatagttaccggataaggcgcagcggtcgggctgaacggggggttcgtgcacacagcccagcttggagcgaacgacctacaccgaactgagatacctacagcgtgagctatgagaaagcgccacgcttcccgaagggagaaaggcggacaggtatccggtaagcggcagggtcggaacaggagagcgcacgagggagcttccagggggaaacgcctggtatctttatagtcctgtcgggtttcgccacctctgacttgagcgtcgatttttgtgatgctcgtcaggggggcggagcctatggaaa

SEQ ID NO: 74 - DNA, 1163 bp, synthetic construct
  source 1..1163: mol_type = other DNA
  misc_feature 1..1163: note = outer region of 5 side of Actinorhodin biosynthetic gene cluster-2
cgataatctagattaattaaatccactccagtacgcgtacgggtgggctgtcctcgggtgccggcaggaggccgcgggccctctcgaacacggcggtcacctgccggccgccctcccgcaccagcccggacagcgcgcgcagggcccgggcggggtccgcgtgcggggtcgggtcgtccgccggggcggtggcccacagcggtacctcgacgatcgccgtggcaccgccgtaccgctggggcgcgcaccaggtggacaggccgatgtcctcggacccggccgccggccgcgcggtgctgcccggcggcggcaggacatggatgccgggggccggattctcccagtacagggcgtcgtacgtgccgtgctggaccgggacccccagggcggcggcggacgccgcgaagggggcggcgagtccggggaggtcgcgggtcagctgggcccaggtgccgcccgcgtcgacgttgtgcagggagcactggaggacggggcgcaggtcgtcgatcacgtcgaacagggcacggctctccgggagtggccggccgacgatcggggcccactccggctgctccgcggcgaccgggcggaaggcggcacggtagtacgacgccagggacggggcggggccggccgtcgcggtctcgatgccctcgctcagcgcggcgccgtccgggtcgaggcacaggacgatgtcccaggtgacggcctcggggtcggtcgccggggagcgccggtcgccgcctgcgaccagctccgccagcgccagtgccgtcgcgccgcccaccggctcgtccgggtgcggccgggccaccaccaggacgtgccggggtccgtggcccaccgacagcatcaggagcggccggcccgcccgggacgtgccgacacgacacaggcggccggtgcccgggaaacgggagaccagccgtcgcgccgactcggtgacctccgcgaccgtggggtatcggttcatcgggcgtgtccggtcaggctccgccgttgccgctctcgtccgccatgccgtctccttccgacggtgcccgtgggtacccgtgggtacctgtgctgcttttcgcgcctgtgctgcctgtggtgtgcgaggcgcgtcgtgccgctgtcagcgtccgttcaccggatcaccgctgtcaatggatcagctcgcg

SEQ ID NO: 75 - DNA, 1107 bp, synthetic construct
  source 1..1107: mol_type = other DNA
  misc_feature 1..1107: note = outer region of 3 side of Actinorhodin biosynthetic gene cluster-2
ccgctgtcaatggatcagctcgcggaggatgtcggcgtggccggcgtggcggccggtctcctccaccatgtgggtgagggcccagcggacactgggcgcggggcggcccggtcgcggccgggggagcggtgcgccgaggtcggtgcaggcgtcgagcacgcggttcgcccgttcgacggcctcccggtagcgggcgacgacgtcggcgacgccgtcctgggacgcggcccggaacgtcgccggccagcttcgcacctcctccccgaggaagaccgcgcgctcgacgtgggtcaggtggttgagcagcccgagcaggttggtgccggacgccaccgccgccgtgcggacctgcggttcgggggcgtcctcgaccttgccggcgatcgaggtccgcaggtagtcgaggaacccgcgcagggtctcggcctcaccgccgccggttcggggcggcggggtgtcccggcggtgggtgcggggggtggtgggcatggtgaccggcctccggaaggtgtggggcgggcgggccgcgggcgcggggcccgtcagtccgcgcggcggacgagcaggacgtggtcgacgacctcggcggtgcgcccgcccgggccggtcgcggtccggcgtggcgcctcggcccgttcgacccgccacgtcgccgggtccagggcgaggtccgccgcgacctcctgcggggccgggtggcgcgcgtcggggtcctggtcccacgaccacggcgccgtcgagccgtggtcgacgaccagcagccgcccgcccgggcgcagcgcgtgcgcggccccgcgcaggaccgacgcgcggtccaggtcgaagggcgtgtggaggtagtgcgcgctgaccaggtcgaaccggccctcggggaaggagtcgcgcaggtcgtgccgcacggcgtcgaccaggtcgccgaggccgtgggtccgtgcgtgccccgcgagccgctcggccgcgaccccggagatgtccacggccgtgacccgccagccccgccgggcaagccacagcgcgtcgccgccgctgccgcaccccaggtccagggcgtcgccgggcggcaggccggtgaccgtctcgaccaggcggacgttcgcatgcctgcag

SEQ ID NO: 76 - DNA, 41 bp, synthetic construct
  source 1..41: mol_type = other DNA
  misc_feature 1..41: note = sco5071-5092del-left-F2
cgataatctagattaattaaatccactccagtacgcgtacg

SEQ ID NO: 77 - DNA, 33 bp, synthetic construct
  source 1..33: mol_type = other DNA
  misc_feature 1..33: note = sco5071-5092del-right-R2
ctgcaggcatgcgaacgtccgcctggtcgagac

SEQ ID NO: 78 - DNA, 8208 bp, synthetic construct
  source 1..8208: mol_type = other DNA
  misc_feature 1..8208: note = pELIM-delta act1
gacggatcttttccgctgcataaccctgcttcggggtcattatagcgattttttcggtatatccatcctttttcgcacgatatacaggattttgccaaagggttcgtgtagactttccttggtgtatccaacggcgtcagccgggcaggataggtgaagtaggcccacccgcgagcgggtgttccttcttcactgtcccttattcgcacctggcggtgctcaacgggaatcctgctctgcgaggctggccggctaccgccggcgtaacagatgagggcaagcggatggctgatgaaaccaagccaaccaggaagggcagcccacctatcaaggtgtactgccttccagacgaacgaagagcgattgaggaaaaggcggcggcggccggcatgagcctgtcggcctacctgctggccgtcggccagggctacaaaatcacgggcgtcgtggactatgagcacgtccgcgagctggcccgcatcaatggcgacctgggccgcctgggcggcctgctgaaactctggctcaccgacgacccgcgcacggcgcggttcggtgatgccacgatcctcgccctgctggcgaagatcgaagagaagcaggacgagcttggcaaggtcatgatgggcgtggtccgcccgagggcagagccatgacttttttagccgctaaaacggccggggggtgcgcgtgattgccaagcacgtccccatgcgctccatcaagaagagcgacttcgcggagctggtgaagtacatcaccgacgagcaaggcaagaccgatccccggggacctgcaggtcgactctagctagcctactgggctgcttcctaatgcaggagtcgcataagggagagcgtcgagatcccggacaccatcgaatggcgcaaaacctttcgcggtatggcatgatagcgcccggaagagagtcaattcagggtggtgaatgtgaaaccagtaacgttatacgatgtcgcagagtatgccggtgtctcttatcagaccgtttcccgcgtggtgaaccaggccagccacgtttctgcgaaaacgcgggaaaaagtggaagcggcgatggcggagctgaattacattcccaaccgcgtggcacaacaactggcgggcaaacagtcgttgctgattggcgttgccacctccagtctggccctgcacgcgccgtcgcaaattgtcgcggcgattaaatctcgcgccgatcaactgggtgccagcgtggtggtgtcgatggtagaacgaagcggcgtcgaagcctgtaaagcggcggtgcacaatcttctcgcgcaacgcgtcagtgggctgatcattaactatccgctggatgaccaggatgccattgctgtggaagctgcctgcactaatgttccggcgttatttcttgatgtctctgaccagacacccatcaacagtattattttctcccatgaagacggtacgcgactgggcgtggagcatctggtcgcattgggtcaccagcaaatcgcgctgttagcgggcccattaagttctgtctcggcgcgtctgcgtctggctggctggcataaatatctcactcgcaatcaaattcagccgatagcggaacgggaaggcgactggagtgccatgtccggttttcaacaaaccatgcaaatgctgaatgagggcatcgttcccactgcgatgctggttgccaacgatcagatggcgctgggcgcaatgcgcgccattaccgagtccgggctgcgcgttggtgcggatatctcggtagtgggatacgacgataccgaagacagctcatgttatatcccgccgttaaccaccatcaaacaggattttcgcctgctggggcaaaccagcgtggaccgcttgctgcaactctctcagggccaggcggtgaagggcaatcagctgttgcccgtctcactggtgaaaagaaaaaccaccctggcgcccaatacgcaaaccgcctctccccgcgcgttggccgattcattaatgcagctggcacgacaggtttcccgactggaaagcgggcagtgagcgcaacgcaattaatgtaagttagctcactcattaggcaccgggatctcggctagctggccagggcccgatacgtcgcggtgagttcaggctttttcatatctcattgcccccggacgagcgtctgctccgccattcgccgtccgccgtgccaatcggatcagccgtccaaatgcgggattttcgttagtcggaggccaaacggcattgagcgtcagcatatcatcagcgagctgaagaaagacaatccccgatccgctccacgtgttgccccagcaatcagcgcgaccttgcccctccaacgtcatctcgttctccgctcatgagctcagccaatcgactggcgagcggcatcgcattcttcgcatcccgcctctggcggatgcaggaagatcaacggatctcggcccagttgacccagggctgtcgccacaatgtcgcgggagcggatcaaccgagcaaaggcatgaccgactggaccttccttctgaaggctcttctccttgagccacctgtccgccaaggcaaagcgctcacagcagtggtcattctcgagataatcgacgcgtaccaacttgccatcctgaagaatggtgcagtgtctcggcaccccatagggaacctttgccatcaactcggcaagatgcagcgtcgtgttggcatcgtgtcccacgccgaggagaagtacctgcccatcgagttcatggacacgggcgaccgggcttgcaggcgagtgaggtggcaggggcaatggatcagagatgatctgctctgcctgtggccccgctgccgcaaaggcaaatggatgggcgctgcgctttacatttggcaggcgccagaatgtgtcagagacaactccaaggtccggtgtaacgggcgacgtggcaggatcgaacggctcgtcgtccagacctgaccacgagggcatgacgagcgtccctcccggacccagcgcagcacgcagggcctcgatcagtccaagtggcccatcttcgaggggccggacgctacggaaggagctgtggaccagcagcacaccgccgggggtaaccccaaggttgagaagctgaccgatgagctcggcttttcgccattcgtattgcacgacattgcactccaccgctgatgacatcagtcgatcatagcacgatcaacggcactgttgcaaatagtcggtggtgataaacttatcatccccttttgctgatggagctgcacatgaaccaaaaggatctaggtgaagatcctttttgataatctcatgaccaaaatcccttaacgtgagttttcgttccactgagcgtcagaccccgtagaaaagatcaaaggatcttcttgagatcctttttttctgcgcgtaatctgctgcttgcaaacaaaaaaaccaccgctaccagcggtggtttgtttgccggatcaagagctaccaactctttttccgaaggtaactggcttcagcagagcgcagataccaaatactgttcttctagtgtagccgtagttaggccaccacttcaagaactctgtagcaccgcctacatacctcgctctgctaatcctgttaccagtggctgctgccagtggcgataagtcgtgtcttaccgggttggactcaagacgatagttaccggataaggcgcagcggtcgggctgaacggggggttcgtgcacacagcccagcttggagcgaacgacctacaccgaactgagatacctacagcgtgagctatgagaaagcgccacgcttcccgaagggagaaaggcggacaggtatccggtaagcggcagggtcggaacaggagagcgcacgagggagcttccagggggaaacgcctggtatctttatagtcctgtcgggtttcgccacctctgacttgagcgtcgatttttgtgatgctcgtcaggggggcggagcctatggaaaaacgccagcaacgcggcctttttacggttcctggccttttgctggccttttgctcacatgttctttcctgcgttatcccctgattctgtggataaccgtattaccgcctttgagtgagctgataccgctcgccgcagccgaacgaccgagcgcagcgagtcagtgagcgaggaagcggaagagcgcccaatacgcaaaccgcctctccccgcgcgttggccgattcattaatgcagctggcacgacaggtttcccgactggaaagcgggcagtgagcgcaacgcaattaatgtgagttagctcactcattaggcaccccaggctttacactttatgcttccggctcgtatgttgtgtggaattgtgagcggataacaatttcacacaggaaacagctatgacatgattacgaattcgatatcagggctacgctggaccggatgggctgagggagccgacggcacgcggcggctcacggcgtggcacgcggaacgtccgggcttgcacctcacgtcacgtgaggaggcagcgtggacggaattgtgagcggataacaattccggcgtcagagaagggagcggagcatatgacgcagtgcccgcgctgccagcggaacctcgcggccgacgagttctacgccgggtcctccaagatgtgcaaggggtgcatgacgtggcagaacctcagctacaacgcgaacaaggaaggccacgcgaacacgttcaccaaggccaccttcctggcctggtacgggctgtccgcgcagcggcactgcgggtactgcgggatctccgaagcggggttcacctccctccaccggacgaacccgcgggggtaccacatccagtgcctgggcgtggaccgctccgacagcttcgagggctactccccccagaacgcccgcctcgcctgcttcatctgcaaccggatcaagagcaacatcttctcggcgtccgagatggacgtgctcggggaggccatctcgaaggcgtggcacgggcgggggatcgcctagagatctccaatatgcggggatcgaccgcgcgggtcccggacggggaagagcggggagctttgccagagagcgacgacttccccttgcgttggtgattgccggtcagggcagccatccgccatcgtcgcgtagggtgtcacaccccaggaatcgcgtcactgaacacagcagccggtaggacgaccatgactgagttggacaccatcgcaaatccgtccgatcccgcggtgcagcggatcatcgatgtcaccaagccgtcgcgatccaacataaagacaacgttgatcgaggacgtcgagcccctcatgcacagcatcgcggccggggtggagttcatcgaggtctacggcagcgacagcagtccttttccatctgagttgctggatctgtgcgggcggcagaacataccggtccgcctcatcgactcctcgatcgtcaaccagttgttcaagggggagcggaaggccaagacattcggcatcgcccgcgtccctcgcccggccaggttcggcgatatcgcgagccggcgtggggacgtcgtcgttctcgacggggtgaagatcgtcgggaacatcggcgcgatagtacgcacgtcgctcgcgctcggagcgtcggggatcatcctggtcgacagtgacatcaccagcatcgcggaccggcgtctccaaagggccagccgaggttacgtcttctcccttcccgtcgttctctccggtcgcgaggaggccatcgccttcattcgggacagcggtatgcagctgatgacgctcaaggcggatggcgacatttccgtgaaggaactcggggacaatccggatcggctggccttgctgttcggcagcgaaaagggtgggccttccgacctgttcgaggaggcgtcttccgcctcggtttccatccccatgatgagccagaccgagtctctcaacgtttccgtttccctcggaatcgcgctgcacgagaggatcgacaggaatctcgcggccaaccgataatctagattaattaaatccactccagtacgcgtacgggtgggctgtcctcgggtgccggcaggaggccgcgggccctctcgaacacggcggtcacctgccggccgccctcccgcaccagcccggacagcgcgcgcagggcccgggcggggtccgcgtgcggggtcgggtcgtccgccggggcggtggcccacagcggtacctcgacgatcgccgtggcaccgccgtaccgctggggcgcgcaccaggtggacaggccgatgtcctcggacccggccgccggccgcgcggtgctgcccggcggcggcaggacatggatgccgggggccggattctcccagtacagggcgtcgtacgtgccgtgctggaccgggacccccagggcggcggcggacgccgcgaagggggcggcgagtccggggaggtcgcgggtcagctgggcccaggtgccgcccgcgtcgacgttgtgcagggagcactggaggacggggcgcaggtcgtcgatcacgtcgaacagggcacggctctccgggagtggccggccgacgatcggggcccactccggctgctccgcggcgaccgggcggaaggcggcacggtagtacgacgccagggacggggcggggccggccgtcgcggtctcgatgccctcgctcagcgcggcgccgtccgggtcgaggcacaggacgatgtcccaggtgacggcctcggggtcggtcgccggggagcgccggtcgccgcctgcgaccagctccgccagcgccagtgccgtcgcgccgcccaccggctcgtccgggtgcggccgggccaccaccaggacgtgccggggtccgtggcccaccgacagcatcaggagcggccggcccgcccgggacgtgccgacacgacacaggcggccggtgcccgggaaacgggagaccagccgtcgcgccgactcggtgacctccgcgaccgtggggtatcggttcatcgggcgtgtccggtcaggctccgccgttgccgctctcgtccgccatgccgtctccttccgacggtgcccgtgggtacccgtgggtacctgtgctgcttttcgcgcctgtgctgcctgtggtgtgcgaggcgcgtcgtgccgctgtcagcgtccgttcaccggatcaccgctgtcaatggatcagctcgcggaggatgtcggcgtggccggcgtggcggccggtctcctccaccatgtgggtgagggcccagcggacactgggcgcggggcggcccggtcgcggccgggggagcggtgcgccgaggtcggtgcaggcgtcgagcacgcggttcgcccgttcgacggcctcccggtagcgggcgacgacgtcggcgacgccgtcctgggacgcggcccggaacgtcgccggccagcttcgcacctcctccccgaggaagaccgcgcgctcgacgtgggtcaggtggttgagcagcccgagcaggttggtgccggacgccaccgccgccgtgcggacctgcggttcgggggcgtcctcgaccttgccggcgatcgaggtccgcaggtagtcgaggaacccgcgcagggtctcggcctcaccgccgccggttcggggcggcggggtgtcccggcggtgggtgcggggggtggtgggcatggtgaccggcctccggaaggtgtggggcgggcgggccgcgggcgcggggcccgtcagtccgcgcggcggacgagcaggacgtggtcgacgacctcggcggtgcgcccgcccgggccggtcgcggtccggcgtggcgcctcggcccgttcgacccgccacgtcgccgggtccagggcgaggtccgccgcgacctcctgcggggccgggtggcgcgcgtcggggtcctggtcccacgaccacggcgccgtcgagccgtggtcgacgaccagcagccgcccgcccgggcgcagcgcgtgcgcggccccgcgcaggaccgacgcgcggtccaggtcgaagggcgtgtggaggtagtgcgcgctgaccaggtcgaaccggccctcggggaaggagtcgcgcaggtcgtgccgcacggcgtcgaccaggtcgccgaggccgtgggtccgtgcgtgccccgcgagccgctcggccgcgaccccggagatgtccacggccgtgacccgccagccccgccgggcaagccacagcgcgtcgccgccgctgccgcaccccaggtccagggcgtcgccgggcggcaggccggtgaccgtctcgaccaggcggacgttcgcatgcctgcaggtc